European Patent Application EP 4 435 112 A2, published September 25, 2024. Title: COMPOSITIONS AND METHODS FOR SCREENING SOLID TUMORS. Applicant: QUEST DIAGNOSTICS INVESTMENTS INCORPORATED. Application US PCT/US2015/057733, filed October 28, 2015. The sequence listing filed with the application follows.

SEQUENCE LISTING (464 sequences)

SEQ ID NO: 1 - DNA, 23 bp, synthetic construct
  misc_feature 1..23: note = Description of Artificial Sequence: Synthetic primer
  source 1..23: mol_type = other DNA
cctagtagaatgtttactaccaa

SEQ ID NO: 2 - DNA, 20 bp, synthetic construct
  misc_feature 1..20: note = Description of Artificial Sequence: Synthetic primer
  source 1..20: mol_type = other DNA
ctgcttcttgagtaacactt

SEQ ID NO: 3 - DNA, 20 bp, synthetic construct
  misc_feature 1..20: note = Description of Artificial Sequence: Synthetic primer
  source 1..20: mol_type = other DNA
catgttcatgctgtgtatgt

SEQ ID NO: 4 - DNA, 22 bp, synthetic construct
  misc_feature 1..22: note = Description of Artificial Sequence: Synthetic primer
  source 1..22: mol_type = other DNA
gcttctttacaaacgttcagaa

SEQ ID NO: 5 - DNA, 21 bp, synthetic construct
  misc_feature 1..21: note = Description of Artificial Sequence: Synthetic primer
  source 1..21: mol_type = other DNA
tctatgttcgaacaggtatct

SEQ ID NO: 6 - DNA, 26 bp, synthetic construct
  misc_feature 1..26: note = Description of Artificial Sequence: Synthetic primer
  source 1..26: mol_type = other DNA
actgctaaacactaatataacctttg

SEQ ID NO: 7 - DNA, 29 bp, synthetic construct
  misc_feature 1..29: note = Description of Artificial Sequence: Synthetic primer
  source 1..29: mol_type = other DNA
ttgaaatgtgttttataatttagactagt

SEQ ID NO: 8 - DNA, 16 bp, synthetic construct
  misc_feature 1..16: note = Description of Artificial Sequence: Synthetic primer
  source 1..16: mol_type = other DNA
ccatgaggtactggcc

SEQ ID NO: 9 - DNA, 21 bp, synthetic construct
  misc_feature 1..21: note = Description of Artificial Sequence: Synthetic primer
  source 1..21: mol_type = other DNA
ttggtgttactggatcaaatc

SEQ ID NO: 10 - DNA, 18 bp, synthetic construct
  misc_feature 1..18: note = Description of Artificial Sequence: Synthetic primer
  source 1..18: mol_type = other DNA
tgctgaaccagtcaaact

SEQ ID NO: 11 - DNA, 31 bp, synthetic construct
  misc_feature 1..31: note = Description of Artificial Sequence: Synthetic primer
  source 1..31: mol_type = other DNA
tattattttattttacagagtaacagactag

SEQ ID NO: 12 - DNA, 20 bp, synthetic construct
  misc_feature 1..20: note = Description of Artificial Sequence: Synthetic primer
  source 1..20: mol_type = other DNA
tttagcacttacctgtgact

SEQ ID NO: 13 - DNA, 18 bp, synthetic construct
  misc_feature 1..18: note = Description of Artificial Sequence: Synthetic primer
  source 1..18: mol_type = other DNA
tggaatgccagaactaca

SEQ ID NO: 14 - DNA, 21 bp, synthetic construct
  misc_feature 1..21: note = Description of Artificial Sequence: Synthetic primer
  source 1..21: mol_type = other DNA
gtggaagatccaatccatttt

SEQ ID NO: 15 - DNA, 21 bp, synthetic construct
  misc_feature 1..21: note = Description of Artificial Sequence: Synthetic primer
  source 1..21: mol_type = other DNA
ggaatgaatggctgaattatg

SEQ ID NO: 16 - DNA, 20 bp, synthetic construct
  misc_feature 1..20: note = Description of Artificial Sequence: Synthetic primer
  source 1..20: mol_type = other DNA
gcggtataatcaggagtttt

SEQ ID NO: 17 - DNA, 20 bp, synthetic construct
  misc_feature 1..20: note = Description of Artificial Sequence: Synthetic primer
  source 1..20: mol_type = other DNA
agttggcctgaatcactata

SEQ ID NO: 18 - DNA, 23 bp, synthetic construct
  misc_feature 1..23: note = Description of Artificial Sequence: Synthetic primer
  source 1..23: mol_type = other DNA
gatgttactattgtgacgatctc

SEQ ID NO: 19 - DNA, 20 bp, synthetic construct
  misc_feature 1..20: note = Description of Artificial Sequence: Synthetic primer
  source 1..20: mol_type = other DNA
gtaagtgttactcaagaagc

SEQ ID NO: 20 - DNA, 27 bp, synthetic construct
  misc_feature 1..27: note = Description of Artificial Sequence: Synthetic primer
  source 1..27: mol_type = other DNA
ataggatattgtatcataccaatttct

SEQ ID NO: 21 - DNA, 20 bp, synthetic construct
  misc_feature 1..20: note = Description of Artificial Sequence: Synthetic primer
  source 1..20: mol_type = other DNA
tccacagctacaccatatat

SEQ ID NO: 22 - DNA, 20 bp, synthetic construct
  misc_feature 1..20: note = Description of Artificial Sequence: Synthetic primer
  source 1..20: mol_type = other DNA
agcatcagcatttgacttta

SEQ ID NO: 23 - DNA, 22 bp, synthetic construct
  misc_feature 1..22: note = Description of Artificial Sequence: Synthetic primer
  source 1..22: mol_type = other DNA
tacacagacactctagtatctg

SEQ ID NO: 24 - DNA, 20 bp, synthetic construct
  misc_feature 1..20: note = Description of Artificial Sequence: Synthetic primer
  source 1..20: mol_type = other DNA
gaaggtttgactgccataaa

SEQ ID NO: 25 - DNA, 20 bp, synthetic construct
  misc_feature 1..20: note = Description of Artificial Sequence: Synthetic primer
  source 1..20: mol_type = other DNA
atgacaaagaacagctcaaa

SEQ ID NO: 26 - DNA, 20 bp, synthetic construct
  misc_feature 1..20: note = Description of Artificial Sequence: Synthetic primer
  source 1..20: mol_type = other DNA
gagatcagccaaattcagtt

SEQ ID NO: 27 - DNA, 22 bp, synthetic construct
  misc_feature 1..22: note = Description of Artificial Sequence: Synthetic primer
  source 1..22: mol_type = other DNA
gatgtgttacaaggcttatcta

SEQ ID NO: 28 - DNA, 20 bp, synthetic construct
  misc_feature 1..20: note = Description of Artificial Sequence: Synthetic primer
  source 1..20: mol_type = other DNA
gcctcttgctcagttttatc

SEQ ID NO: 29 - DNA, 19 bp, synthetic construct
  misc_feature 1..19: note = Description of Artificial Sequence: Synthetic primer
  source 1..19: mol_type = other DNA
gaggctttggagtatttca

SEQ ID NO: 30 - DNA, 21 bp, synthetic construct
  misc_feature 1..21: note = Description of Artificial Sequence: Synthetic primer
  source 1..21: mol_type = other DNA
ctgctgagagttattaacagt

SEQ ID NO: 31 - DNA, 19 bp, synthetic construct
  misc_feature 1..19: note = Description of Artificial Sequence: Synthetic primer
  source 1..19: mol_type = other DNA
gcttttggagtcctattgt

SEQ ID NO: 32 - DNA, 20 bp, synthetic construct
  misc_feature 1..20: note = Description of Artificial Sequence: Synthetic primer
  source 1..20: mol_type = other DNA
cacaaactagagtcacacac

SEQ ID NO: 33 - DNA, 19 bp, synthetic construct
  misc_feature 1..19: note = Description of Artificial Sequence: Synthetic primer
  source 1..19: mol_type = other DNA
gggttttgggctgatatta

SEQ ID NO: 34 - DNA, 20 bp, synthetic construct
  misc_feature 1..20: note = Description of Artificial Sequence: Synthetic primer
  source 1..20: mol_type = other DNA
ccacagaactgaaggttaat

SEQ ID NO: 35 - DNA, 31 bp, synthetic construct
  misc_feature 1..31: note = Description of Artificial Sequence: Synthetic primer
  source 1..31: mol_type = other DNA
ttatccattgaatttattttaatctttctag

SEQ ID NO: 36 - DNA, 18 bp, synthetic construct
  misc_feature 1..18: note = Description of Artificial Sequence: Synthetic primer
  source 1..18: mol_type = other DNA
gggatgtgcgggtatatt

SEQ ID NO: 37 - DNA, 20 bp, synthetic construct
  misc_feature 1..20: note = Description of Artificial Sequence: Synthetic primer
  source 1..20: mol_type = other DNA
gtcttgcagtaagagattgt

SEQ ID NO: 38 - DNA, 16 bp, synthetic construct
  misc_feature 1..16: note = Description of Artificial Sequence: Synthetic primer
  source 1..16: mol_type = other DNA
tctttgctgtaccgct

SEQ ID NO: 39 - DNA, 16 bp, synthetic construct
  misc_feature 1..16: note = Description of Artificial Sequence: Synthetic primer
  source 1..16: mol_type = other DNA
gtttcttttgcctgca

SEQ ID NO: 40 - DNA, 21 bp, synthetic construct
  misc_feature 1..21: note = Description of Artificial Sequence: Synthetic primer
  source 1..21: mol_type = other DNA
tggataaggtctggtttaatg

SEQ ID NO: 41 - DNA, 21 bp, synthetic construct
  misc_feature 1..21: note = Description of Artificial Sequence: Synthetic primer
  source 1..21: mol_type = other DNA
gctacaattcaggatgagtta

SEQ ID NO: 42 - DNA, 21 bp, synthetic construct
  misc_feature 1..21: note = Description of Artificial Sequence: Synthetic primer
  source 1..21: mol_type = other DNA
tcttctgctatcaccatcttt

SEQ ID NO: 43 - DNA, 20 bp, synthetic construct
  misc_feature 1..20: note = Description of Artificial Sequence: Synthetic primer
  source 1..20: mol_type = other DNA
ccatcatgatgagaagacat

SEQ ID NO: 44 - DNA, 20 bp, synthetic construct
  misc_feature 1..20: note = Description of Artificial Sequence: Synthetic primer
  source 1..20: mol_type = other DNA
ttgctggagatacatacact

SEQ ID NO: 45 - DNA, 20 bp, synthetic construct
  misc_feature 1..20: note = Description of Artificial Sequence: Synthetic primer
  source 1..20: mol_type = other DNA
gtggtcactaaaccttaaga

SEQ ID NO: 46 - DNA, 20 bp, synthetic construct
  misc_feature 1..20: note = Description of Artificial Sequence: Synthetic primer
  source 1..20: mol_type = other DNA
ggcttaccttagtgtaagag

SEQ ID NO: 47 - DNA, 22 bp, synthetic construct
  misc_feature 1..22: note = Description of Artificial Sequence: Synthetic primer
  source 1..22: mol_type = other DNA
tttcatcgagatgggaaatatg

SEQ ID NO: 48 - DNA, 21 bp, synthetic construct
  misc_feature 1..21: note = Description of Artificial Sequence: Synthetic primer
  source 1..21: mol_type = other DNA
acctgttggtatttggatact

SEQ ID NO: 49 - DNA, 24 bp, synthetic construct
  misc_feature 1..24: note = Description of Artificial Sequence: Synthetic primer
  source 1..24: mol_type = other DNA
agaagataatattgaagctgtagg

SEQ ID NO: 50 - DNA, 29 bp, synthetic construct
  misc_feature 1..29: note = Description of Artificial Sequence: Synthetic primer
  source 1..29: mol_type = other DNA
agaactcttattttttaatctgattttca

SEQ ID NO: 51 - DNA, 21 bp, synthetic construct
  misc_feature 1..21: note = Description of Artificial Sequence: Synthetic primer
  source 1..21: mol_type = other DNA
ggacagctattgaagcattta

SEQ ID NO: 52 - DNA, 20 bp, synthetic construct
  misc_feature 1..20: note = Description of Artificial Sequence: Synthetic primer
  source 1..20: mol_type = other DNA
cacaagaacaagggaaacac

SEQ ID NO: 53 - DNA, 17 bp, synthetic construct
  misc_feature 1..17: note = Description of Artificial Sequence: Synthetic primer
  source 1..17: mol_type = other DNA
gcaggcagctgagtatc

SEQ ID NO: 54 - DNA, 22 bp, synthetic construct
  misc_feature 1..22: note = Description of Artificial Sequence: Synthetic primer
  source 1..22: mol_type = other DNA
tcatcctgaattgtagcaatca

SEQ ID NO: 55 - DNA, 17 bp, synthetic construct
  misc_feature 1..17: note = Description of Artificial Sequence: Synthetic primer
  source 1..17: mol_type = other DNA
cagcttctgccatctct

SEQ ID NO: 56 - DNA, 15 bp, synthetic construct
  misc_feature 1..15: note = Description of Artificial Sequence: Synthetic primer
  source 1..15: mol_type = other DNA
agcagccgcagaaat

SEQ ID NO: 57 - DNA, 19 bp, synthetic construct
  misc_feature 1..19: note = Description of Artificial Sequence: Synthetic primer
  source 1..19: mol_type = other DNA
gtggctttttgtttgtttg

SEQ ID NO: 58 - DNA, 21 bp, synthetic construct
  misc_feature 1..21: note = Description of Artificial Sequence: Synthetic primer
  source 1..21: mol_type = other DNA
cactctaacaagcagataact

SEQ ID NO: 59 - DNA, 29 bp, synthetic construct
  misc_feature 1..29: note = Description of Artificial Sequence: Synthetic primer
  source 1..29: mol_type = other DNA
tacttgttaattaaaaattcaagagtttt

SEQ ID NO: 60 - DNA, 20 bp, synthetic construct
  misc_feature 1..20: note = Description of Artificial Sequence: Synthetic primer
  source 1..20: mol_type = other DNA
cttagccattggtcaagatc

SEQ ID NO: 61 - DNA, 17 bp, synthetic construct
  misc_feature 1..17: note = Description of Artificial Sequence: Synthetic primer
  source 1..17: mol_type = other DNA
acaatcatgttgcagca

SEQ ID NO: 62 - DNA, 28 bp, synthetic construct
  misc_feature 1..28: note = Description of Artificial Sequence: Synthetic primer
  source 1..28: mol_type = other DNA
aaaaacatcaaaaaataacttacctttt

SEQ ID NO: 63 - DNA, 19 bp, synthetic construct
  misc_feature 1..19: note = Description of Artificial Sequence: Synthetic primer
  source 1..19: mol_type = other DNA
agaggcgctatgtgtatta

SEQ ID NO: 64 - DNA, 21 bp, synthetic construct
  misc_feature 1..21: note = Description of Artificial Sequence: Synthetic primer
  source 1..21: mol_type = other DNA
catggaaggatgagaatttca

SEQ ID NO: 65 - DNA, 20 bp, synthetic construct
  misc_feature 1..20: note = Description of Artificial Sequence: Synthetic primer
  source 1..20: mol_type = other DNA
ggaagacaagttcatgtact

SEQ ID NO: 66 - DNA, 24 bp, synthetic construct
  misc_feature 1..24: note = Description of Artificial Sequence: Synthetic primer
  source 1..24: mol_type = other DNA
ctgtccttattttggatatttctc

SEQ ID NO: 67 - DNA, 32 bp, synthetic construct
  misc_feature 1..32: note = Description of Artificial Sequence: Synthetic primer
  source 1..32: mol_type = other DNA
attaattaaatatgtcatttcatttctttttc

SEQ ID NO: 68 - DNA, 21 bp, synthetic construct
  misc_feature 1..21: note = Description of Artificial Sequence: Synthetic primer
  source 1..21: mol_type = other DNA
gctatcgatttcttgatcaca

SEQ ID NO: 69 - DNA, 22 bp, synthetic construct
  misc_feature 1..22: note = Description of Artificial Sequence: Synthetic primer
  source 1..22: mol_type = other DNA
tgagtcatatttgtgggttttc

SEQ ID NO: 70 - DNA, 22 bp, synthetic construct
  misc_feature 1..22: note = Description of Artificial Sequence: Synthetic primer
  source 1..22: mol_type = other DNA
tgatcaggttcattgtcactaa

SEQ ID NO: 71 - DNA, 21 bp, synthetic construct
  misc_feature 1..21: note = Description of Artificial Sequence: Synthetic primer
  source 1..21: mol_type = other DNA
tttgattgctgcatatttcag

SEQ ID NO: 72 - DNA, 23 bp, synthetic construct
  misc_feature 1..23: note = Description of Artificial Sequence: Synthetic primer
  source 1..23: mol_type = other DNA
tcaaagcattcttaccttactac

SEQ ID NO: 73 - DNA, 25 bp, synthetic construct
  misc_feature 1..25: note = Description of Artificial Sequence: Synthetic primer
  source 1..25: mol_type = other DNA
ttttaaacttttcttttagttgtgc

SEQ ID NO: 74 - DNA, 20 bp, synthetic construct
  misc_feature 1..20: note = Description of Artificial Sequence: Synthetic primer
  source 1..20: mol_type = other DNA
actcgataatctggatgact

SEQ ID NO: 75 - DNA, 28 bp, synthetic construct
  misc_feature 1..28: note = Description of Artificial Sequence: Synthetic primer
  source 1..28: mol_type = other DNA
caatttagtgaaataactataatggaac

SEQ ID NO: 76 - DNA, 19 bp, synthetic construct
  misc_feature 1..19: note = Description of Artificial Sequence: Synthetic primer
  source 1..19: mol_type = other DNA
agtgccactggtctataat

SEQ ID NO: 77 - DNA, 23 bp, synthetic construct
  misc_feature 1..23: note = Description of Artificial Sequence: Synthetic primer
  source 1..23: mol_type = other DNA
cctgtgaaataatactggtatgt

SEQ ID NO: 78 - DNA, 22 bp, synthetic construct
  misc_feature 1..22: note = Description of Artificial Sequence: Synthetic primer
  source 1..22: mol_type = other DNA
ctactttgatatcaccacacac

SEQ ID NO: 79 - DNA, 19 bp, synthetic construct
  misc_feature 1..19: note = Description of Artificial Sequence: Synthetic primer
  source 1..19: mol_type = other DNA
tagagcgtgcagataatga

SEQ ID NO: 80 - DNA, 17 bp, synthetic construct
  misc_feature 1..17: note = Description of Artificial Sequence: Synthetic primer
  source 1..17: mol_type = other DNA
tcaacaacccccacaaa

SEQ ID NO: 81 - DNA, 21 bp, synthetic construct
  misc_feature 1..21: note = Description of Artificial Sequence: Synthetic primer
  source 1..21: mol_type = other DNA
ctttctctaggtgaagctgta

SEQ ID NO: 82 - DNA, 20 bp, synthetic construct
  misc_feature 1..20: note = Description of Artificial Sequence: Synthetic primer
  source 1..20: mol_type = other DNA
ggttcattctctggatcaga

SEQ ID NO: 83 - DNA, 18 bp, synthetic construct
  misc_feature 1..18: note = Description of Artificial Sequence: Synthetic primer
  source 1..18: mol_type = other DNA
ctgaggtggaagagacag

SEQ ID NO: 84 - DNA, 17 bp, synthetic construct
  misc_feature 1..17: note = Description of Artificial Sequence: Synthetic primer
  source 1..17: mol_type = other DNA
actggttctcactcacc

SEQ ID NO: 85 - DNA, 16 bp, synthetic construct
  misc_feature 1..16: note = Description of Artificial Sequence: Synthetic primer
  source 1..16: mol_type = other DNA
gccagcaaagcagtag

SEQ ID NO: 86 - DNA, 21 bp, synthetic construct
  misc_feature 1..21: note = Description of Artificial Sequence: Synthetic primer
  source 1..21: mol_type = other DNA
tggaaaaatagcctcaattct

SEQ ID NO: 87 - DNA, 22 bp, synthetic construct
  misc_feature 1..22: note = Description of Artificial Sequence: Synthetic primer
  source 1..22: mol_type = other DNA
caccacattacatacttaccat

SEQ ID NO: 88 - DNA, 22 bp, synthetic construct
  misc_feature 1..22: note = Description of Artificial Sequence: Synthetic primer
  source 1..22: mol_type = other DNA
ctctggaaaagagtaattcaca

SEQ ID NO: 89 - DNA, 23 bp, synthetic construct
  misc_feature 1..23: note = Description of Artificial Sequence: Synthetic primer
  source 1..23: mol_type = other DNA
cgtatttatagctgatttgatgg

SEQ ID NO: 90 - DNA, 18 bp, synthetic construct
  misc_feature 1..18: note = Description of Artificial Sequence: Synthetic primer
  source 1..18: mol_type = other DNA
ggacttcacctgacagat

SEQ ID NO: 91 - DNA, 21 bp, synthetic construct
  misc_feature 1..21: note = Description of Artificial Sequence: Synthetic primer
  source 1..21: mol_type = other DNA
ctttggtttctcttggtctag

SEQ ID NO: 92 - DNA, 20 bp, synthetic construct
  misc_feature 1..20: note = Description of Artificial Sequence: Synthetic primer
  source 1..20: mol_type = other DNA
gagtttctgcagattgactt

SEQ ID NO: 93 - DNA, 18 bp, synthetic construct
  misc_feature 1..18: note = Description of Artificial Sequence: Synthetic primer
  source 1..18: mol_type = other DNA
gtgtttcctttgcagatg

SEQ ID NO: 94 - DNA, 19 bp, synthetic construct
  misc_feature 1..19: note = Description of Artificial Sequence: Synthetic primer
  source 1..19: mol_type = other DNA
tcacatgcctctttctcta

SEQ ID NO: 95 - DNA, 16 bp, synthetic construct
  misc_feature 1..16: note = Description of Artificial Sequence: Synthetic primer
  source 1..16: mol_type = other DNA
cctggctctgactcac

SEQ ID NO: 96 - DNA, 17 bp, synthetic construct
  misc_feature 1..17: note = Description of Artificial Sequence: Synthetic primer
  source 1..17: mol_type = other DNA
tttccctgccaagtgat

SEQ ID NO: 97 - DNA, 14 bp, synthetic construct
  misc_feature 1..14: note = Description of Artificial Sequence: Synthetic primer
  source 1..14: mol_type = other DNA
tgcagcggtgttgt

SEQ ID NO: 98 - DNA, 15 bp, synthetic construct
  misc_feature 1..15: note = Description of Artificial Sequence: Synthetic primer
  source 1..15: mol_type = other DNA
tctcggctcaaggac

SEQ ID NO: 99 - DNA, 20 bp, synthetic construct
  misc_feature 1..20: note = Description of Artificial Sequence: Synthetic primer
  source 1..20: mol_type = other DNA
ttcctcagttacaccaatct

SEQ ID NO: 100 - DNA, 17 bp, synthetic construct
  misc_feature 1..17: note = Description of Artificial Sequence: Synthetic primer
  source 1..17: mol_type = other DNA
gcctttggggttacttt

SEQ ID NO: 101 - DNA, 18 bp, synthetic construct
  misc_feature 1..18: note = Description of Artificial Sequence: Synthetic primer
  source 1..18: mol_type = other DNA
gctgctggagaagagata

SEQ ID NO: 102 - DNA, 17 bp, synthetic construct
  misc_feature 1..17: note = Description of Artificial Sequence: Synthetic primer
  source 1..17: mol_type = other DNA
aggtggctggttatgtc

SEQ ID NO: 103 - DNA, 21 bp, synthetic construct
  misc_feature 1..21: note = Description of Artificial Sequence: Synthetic primer
  source 1..21: mol_type = other DNA
ggagataagtgatggagatgt

SEQ ID NO: 104 - DNA, 16 bp, synthetic construct
  misc_feature 1..16: note = Description of Artificial Sequence: Synthetic primer
  source 1..16: mol_type = other DNA
ggatcggcctcttcat

SEQ ID NO: 105 - DNA, 17 bp, synthetic construct
  misc_feature 1..17: note = Description of Artificial Sequence: Synthetic primer
  source 1..17: mol_type = other DNA
cccaaccaagctctctt

SEQ ID NO: 106 - DNA, 15 bp, synthetic construct
  misc_feature 1..15: note = Description of Artificial Sequence: Synthetic primer
  source 1..15: mol_type = other DNA
actgacgtgcctctc

SEQ ID NO: 107 - DNA, 17 bp, synthetic construct
  misc_feature 1..17: note = Description of Artificial Sequence: Synthetic primer
  source 1..17: mol_type = other DNA
gcagggtcttctctgtt

SEQ ID NO: 108 - DNA, 21 bp, synthetic construct
  misc_feature 1..21: note = Description of Artificial Sequence: Synthetic primer
  source 1..21: mol_type = other DNA
ccaacagagggaaactaatag

SEQ ID NO: 109 - DNA, 18 bp, synthetic construct
  misc_feature 1..18: note = Description of Artificial Sequence: Synthetic primer
  source 1..18: mol_type = other DNA
ctgatggggagaatgtga

SEQ ID NO: 110 - DNA, 20 bp, synthetic construct
  misc_feature 1..20: note = Description of Artificial Sequence: Synthetic primer
  source 1..20: mol_type = other DNA
catttgaccatgaccatgta

SEQ ID NO: 111 - DNA, 20 bp, synthetic construct
  misc_feature 1..20: note = Description of Artificial Sequence: Synthetic primer
  source 1..20: mol_type = other DNA
cccatgaataccagtgacta

SEQ ID NO: 112 - DNA, 20 bp, synthetic construct
  misc_feature 1..20: note = Description of Artificial Sequence: Synthetic primer
  source 1..20: mol_type = other DNA
ctgttacttacgtggacatt

SEQ ID NO: 113 - DNA, 19 bp, synthetic construct
  misc_feature 1..19: note = Description of Artificial Sequence: Synthetic primer
  source 1..19: mol_type = other DNA
ctcattcatcgccacatag

SEQ ID NO: 114 - DNA, 20 bp, synthetic construct
  misc_feature 1..20: note = Description of Artificial Sequence: Synthetic primer
  source 1..20: mol_type = other DNA
gacttaccttgcaatgtttg

SEQ ID NO: 115 - DNA, 18 bp, synthetic construct
  misc_feature 1..18: note = Description of Artificial Sequence: Synthetic primer
  source 1..18: mol_type = other DNA
actggcctgtctcaatat

SEQ ID NO: 116 - DNA, 20 bp, synthetic construct
  misc_feature 1..20: note = Description of Artificial Sequence: Synthetic primer
  source 1..20: mol_type = other DNA
agtggaagtatgcccatata

SEQ ID NO: 117 - DNA, 21 bp, synthetic construct
  misc_feature 1..21: note = Description of Artificial Sequence: Synthetic primer
  source 1..21: mol_type = other DNA
tacagaagaggagtgtcatat

SEQ ID NO: 118 - DNA, 16 bp, synthetic construct
  misc_feature 1..16: note = Description of Artificial Sequence: Synthetic primer
  source 1..16: mol_type = other DNA
tgcccactgtgttact

SEQ ID NO: 119 - DNA, 21 bp, synthetic construct
  misc_feature 1..21: note = Description of Artificial Sequence: Synthetic primer
  source 1..21: mol_type = other DNA
agttgtgggtacctttagatt

SEQ ID NO: 120 - DNA, 12 bp, synthetic construct
  misc_feature 1..12: note = Description of Artificial Sequence: Synthetic primer
  source 1..12: mol_type = other DNA
ggcggtggtggt

SEQ ID NO: 121 - DNA, 14 bp, synthetic construct
  misc_feature 1..14: note = Description of Artificial Sequence: Synthetic primer
  source 1..14: mol_type = other DNA
gccaggcctcaacg

SEQ ID NO: 122 - DNA, 15 bp, synthetic construct
  misc_feature 1..15: note = Description of Artificial Sequence: Synthetic primer
  source 1..15: mol_type = other DNA
gtgaccgaggacaac

SEQ ID NO: 123 - DNA, 15 bp, synthetic construct
  misc_feature 1..15: note = Description of Artificial Sequence: Synthetic primer
  source 1..15: mol_type = other DNA
ctgaccgacgttgac

SEQ ID NO: 124 - DNA, 17 bp, synthetic construct
  misc_feature 1..17: note = Description of Artificial Sequence: Synthetic primer
  source 1..17: mol_type = other DNA
cctgggattgcagattg

SEQ ID NO: 125 - DNA, 20 bp, synthetic construct
  misc_feature 1..20: note = Description of Artificial Sequence: Synthetic primer
  source 1..20: mol_type = other DNA
gtttcatggactcagttact

SEQ ID NO: 126 - DNA, 20 bp, synthetic construct
  misc_feature 1..20: note = Description of Artificial Sequence: Synthetic primer
  source 1..20: mol_type = other DNA
ccagacctttgctttagatt

SEQ ID NO: 127 - DNA, 20 bp, synthetic construct
  misc_feature 1..20: note = Description of Artificial Sequence: Synthetic primer
  source 1..20: mol_type = other DNA
aaagacttggtgttgttgat

SEQ ID NO: 128 - DNA, 20 bp, synthetic construct
  misc_feature 1..20: note = Description of Artificial Sequence: Synthetic primer
  source 1..20: mol_type = other DNA
gcccatcatatttcttcaga

SEQ ID NO: 129 - DNA, 17 bp, synthetic construct
  misc_feature 1..17: note = Description of Artificial Sequence: Synthetic primer
  source 1..17: mol_type = other DNA
cgtgccacccagaatat

SEQ ID NO: 130 - DNA, 14 bp, synthetic construct
  misc_feature 1..14: note = Description of Artificial Sequence: Synthetic primer
  source 1..14: mol_type = other DNA
ggcctacctggtcg

SEQ ID NO: 131 - DNA, 19 bp, synthetic construct
  misc_feature 1..19: note = Description of Artificial Sequence: Synthetic primer
  source 1..19: mol_type = other DNA
ttccagcactctgacatat

SEQ ID NO: 132 - DNA, 16 bp, synthetic construct
  misc_feature 1..16: note = Description of Artificial Sequence: Synthetic primer
  source 1..16: mol_type = other DNA
tgcttttagggcccac

SEQ ID NO: 133 - DNA, 22 bp, synthetic construct
  misc_feature 1..22: note = Description of Artificial Sequence: Synthetic primer
  source 1..22: mol_type = other DNA
ccaacctaatagtgtattcaca

SEQ ID NO: 134 - DNA, 20 bp, synthetic construct
  misc_feature 1..20: note = Description of Artificial Sequence: Synthetic primer
  source 1..20: mol_type = other DNA
attattgactctgttgtgct

SEQ ID NO: 135 - DNA, 17 bp, synthetic construct
  misc_feature 1..17: note = Description of Artificial Sequence: Synthetic primer
  source 1..17: mol_type = other DNA
ccccagtcctcatgtac

SEQ ID NO: 136 - DNA, 16 bp, synthetic construct
  misc_feature 1..16: note = Description of Artificial Sequence: Synthetic primer
  source 1..16: mol_type = other DNA
gctggaggagctagag

SEQ ID NO: 137 - DNA, 20 bp, synthetic construct
  misc_feature 1..20: note = Description of Artificial Sequence: Synthetic primer
  source 1..20: mol_type = other DNA
ccttctcttccccaatctac

SEQ ID NO: 138 - DNA, 16 bp, synthetic construct
  misc_feature 1..16: note = Description of Artificial Sequence: Synthetic primer
  source 1..16: mol_type = other DNA
aggagccaggcatttt

SEQ ID NO: 139 - DNA, 20 bp, synthetic construct
  misc_feature 1..20: note = Description of Artificial Sequence: Synthetic primer
  source 1..20: mol_type = other DNA
ctttccccacaatcatactg

SEQ ID NO: 140 - DNA, 19 bp, synthetic construct
  misc_feature 1..19: note = Description of Artificial Sequence: Synthetic primer
  source 1..19: mol_type = other DNA
gctggtgttgtctcaatat

SEQ ID NO: 141 - DNA, 19 bp, synthetic construct
  misc_feature 1..19: note = Description of Artificial Sequence: Synthetic primer
  source 1..19: mol_type = other DNA
tacgatgcaagagtacaca

SEQ ID NO: 142 - DNA, 18 bp, synthetic construct
  misc_feature 1..18: note = Description of Artificial Sequence: Synthetic primer
  source 1..18: mol_type = other DNA
ccaccactggatttctca

SEQ ID NO: 143 - DNA, 20 bp, synthetic construct
  misc_feature 1..20: note = Description of Artificial Sequence: Synthetic primer
  source 1..20: mol_type = other DNA
cttattggctttggtcttca

SEQ ID NO: 144 - DNA, 27 bp, synthetic construct
  misc_feature 1..27: note = Description of Artificial Sequence: Synthetic primer
  source 1..27: mol_type = other DNA
tcagcatcattgtaaattattctattt

SEQ ID NO: 145 - DNA, 15 bp, synthetic construct
  misc_feature 1..15: note = Description of Artificial Sequence: Synthetic primer
  source 1..15: mol_type = other DNA
acgagctggaccact

SEQ ID NO: 146 - DNA, 15 bp, synthetic construct
  misc_feature 1..15: note = Description of Artificial Sequence: Synthetic primer
  source 1..15: mol_type = other DNA
tcggctctccactca

SEQ ID NO: 147 - DNA, 16 bp, synthetic construct
  misc_feature 1..16: note = Description of Artificial Sequence: Synthetic primer
  source 1..16: mol_type = other DNA
gggccacacttactct

SEQ ID NO: 148 - DNA, 14 bp, synthetic construct
  misc_feature 1..14: note = Description of Artificial Sequence: Synthetic primer
  source 1..14: mol_type = other DNA
ccgggtctcactca

SEQ ID NO: 149 - DNA, 20 bp, synthetic construct
  misc_feature 1..20: note = Description of Artificial Sequence: Synthetic primer
  source 1..20: mol_type = other DNA
cgtagtaggggaagatcatc

SEQ ID NO: 150 - DNA, 17 bp, synthetic construct
  misc_feature 1..17: note = Description of Artificial Sequence: Synthetic primer
  source 1..17: mol_type = other DNA
ggacactcgcagtagaa

SEQ ID NO: 151 - DNA, 22 bp, synthetic construct
  misc_feature 1..22: note = Description of Artificial Sequence: Synthetic primer
  source 1..22: mol_type = other DNA
ataatgctcctagtacctgtag

SEQ ID NO: 152 - DNA, 19 bp, synthetic construct
  misc_feature 1..19: note = Description of Artificial Sequence: Synthetic primer
  source 1..19: mol_type = other DNA
cttgcacaaatgctgaaag

SEQ ID NO: 153 - DNA, 23 bp, synthetic construct
  misc_feature 1..23: note = Description of Artificial Sequence: Synthetic primer
  source 1..23: mol_type = other DNA
catttatagaaaccgaggtatga

SEQ ID NO: 154 - DNA, 18 bp, synthetic construct
  misc_feature 1..18: note = Description of Artificial Sequence: Synthetic primer
  source 1..18: mol_type = other DNA
gtctgcaggacaattcat

SEQ ID NO: 155 - DNA, 20 bp, synthetic construct
  misc_feature 1..20: note = Description of Artificial Sequence: Synthetic primer
  source 1..20: mol_type = other DNA
tccacaaagccccttataat

SEQ ID NO: 156 - DNA, 19 bp, synthetic construct
  misc_feature 1..19: note = Description of Artificial Sequence: Synthetic primer
  source 1..19: mol_type = other DNA
cttgtttcaggcatgtagt

SEQ ID NO: 157 - DNA, 14 bp, synthetic construct
  misc_feature 1..14: note = Description of Artificial Sequence: Synthetic primer
  source 1..14: mol_type = other DNA
cccacgccgtctta

SEQ ID NO: 158 - DNA, 16 bp, synthetic construct
  misc_feature 1..16: note = Description of Artificial Sequence: Synthetic primer
  source 1..16: mol_type = other DNA
agcggtggtgtagtac

SEQ ID NO: 159 - DNA, 17 bp, synthetic construct
  misc_feature 1..17: note = Description of Artificial Sequence: Synthetic primer
  source 1..17: mol_type = other DNA
aagtgccttagcagaga

SEQ ID NO: 160 - DNA, 20 bp, synthetic construct
  misc_feature 1..20: note = Description of Artificial Sequence: Synthetic primer
  source 1..20: mol_type = other DNA
agacatcagaaagcatgatc

SEQ ID NO: 161 - DNA, 17 bp, synthetic construct
  misc_feature 1..17: note = Description of Artificial Sequence: Synthetic primer
  source 1..17: mol_type = other DNA
ccatgaggcagagcata

SEQ ID NO: 162 - DNA, 14 bp, synthetic construct
  misc_feature 1..14: note = Description of Artificial Sequence: Synthetic primer
  source 1..14: mol_type = other DNA
ggccatggcctgac

SEQ ID NO: 163 - DNA, 17 bp, synthetic construct
  misc_feature 1..17: note = Description of Artificial Sequence: Synthetic primer
  source 1..17: mol_type = other DNA
tatggtcatggaagggg

SEQ ID NO: 164 - DNA, 13 bp, synthetic construct
  misc_feature 1..13: note = Description of Artificial Sequence: Synthetic primer
  source 1..13: mol_type = other DNA
ccgctgagccact

SEQ ID NO: 165 - DNA, 19 bp, synthetic construct
  misc_feature 1..19: note = Description of Artificial Sequence: Synthetic primer
  source 1..19: mol_type = other DNA
gcgtcatcatctttgtcat

SEQ ID NO: 166 - DNA, 18 bp, synthetic construct
  misc_feature 1..18: note = Description of Artificial Sequence: Synthetic primer
  source 1..18: mol_type = other DNA
catccctgactgtgagat

SEQ ID NO: 167 - DNA, 15 bp, synthetic construct
  misc_feature 1..15: note = Description of Artificial Sequence: Synthetic primer
  source 1..15: mol_type = other DNA
ggtggcatggacaga

SEQ ID NO: 168 - DNA, 18 bp, synthetic construct
  misc_feature 1..18: note = Description of Artificial Sequence: Synthetic primer
  source 1..18: mol_type = other DNA
gtgggctacaagaactac

SEQ ID NO: 169 - DNA, 18 bp, synthetic construct
  misc_feature 1..18: note = Description of Artificial Sequence: Synthetic primer
  source 1..18: mol_type = other DNA
gggtatggacacgttcat

SEQ ID NO: 170 - DNA, 20 bp, synthetic construct
  misc_feature 1..20: note = Description of Artificial Sequence: Synthetic primer
  source 1..20: mol_type = other DNA
cctcgaaatgaagctacaac

SEQ ID NO: 171 - DNA, 19 bp, synthetic construct
  misc_feature 1..19: note = Description of Artificial Sequence: Synthetic primer
  source 1..19: mol_type = other DNA
aagtggagaatgtcagtct

SEQ ID NO: 172 - DNA, 22 bp, synthetic construct
  misc_feature 1..22: note = Description of Artificial Sequence: Synthetic primer
  source 1..22: mol_type = other DNA
gaaactttccacttgataagag

SEQ ID NO: 173 - DNA, 17 bp, synthetic construct
  misc_feature 1..17: note = Description of Artificial Sequence: Synthetic primer
  source 1..17: mol_type = other DNA
ttacctcgcttagtgct

SEQ ID NO: 174 - DNA, 15 bp, synthetic construct
  misc_feature 1..15: note = Description of Artificial Sequence: Synthetic primer
  source 1..15: mol_type = other DNA
cccagagaccccagt

SEQ ID NO: 175 - DNA, 15 bp, synthetic construct
  misc_feature 1..15: note = Description of Artificial Sequence: Synthetic primer
  source 1..15: mol_type = other DNA
agccctgtcgtctct

SEQ ID NO: 176 - DNA, 16 bp, synthetic construct
  misc_feature 1..16: note = Description of Artificial Sequence: Synthetic primer
  source 1..16: mol_type = other DNA
gccaggcattgaagtc

SEQ ID NO: 177 - DNA, 14 bp, synthetic construct
  misc_feature 1..14: note = Description of Artificial Sequence: Synthetic primer
  source 1..14: mol_type = other DNA
gagctgctggtgca

SEQ ID NO: 178 - DNA, 18 bp, synthetic construct
  misc_feature 1..18: note = Description of Artificial Sequence: Synthetic primer
  source 1..18: mol_type = other DNA
tccaatggatccactcac

SEQ ID NO: 179 - DNA, 19 bp, synthetic construct
  misc_feature 1..19: note = Description of Artificial Sequence: Synthetic primer
  source 1..19: mol_type = other DNA
gcatttcctttcttcccag

SEQ ID NO: 180 - DNA, 19 bp, synthetic construct
  misc_feature 1..19: note = Description of Artificial Sequence: Synthetic primer
  source 1..19: mol_type = other DNA
ttggttacatccctctctg

SEQ ID NO: 181 - DNA, 16 bp, synthetic construct
  misc_feature 1..16: note = Description of Artificial Sequence: Synthetic primer
  source 1..16: mol_type = other DNA
tgttgcagctgaccac

SEQ ID NO: 182 - DNA, 23 bp, synthetic construct
  misc_feature 1..23: note = Description of Artificial Sequence: Synthetic primer
  source 1..23: mol_type = other DNA
tgttttcctttacttactacacc

SEQ ID NO: 183 - DNA, 20 bp, synthetic construct
  misc_feature 1..20: note = Description of Artificial Sequence: Synthetic primer
  source 1..20: mol_type = other DNA
tttggcttgacttgactttt

SEQ ID NO: 184 - DNA, 21 bp, synthetic construct
  misc_feature 1..21: note = Description of Artificial Sequence: Synthetic primer
  source 1..21: mol_type = other DNA
tgaaatgacacttggagtaac

SEQ ID NO: 185 - DNA, 19 bp, synthetic construct
  misc_feature 1..19: note = Description of Artificial Sequence: Synthetic primer
  source 1..19: mol_type = other DNA
gtatccacatcctcttcct

SEQ ID NO: 186 - DNA, 20 bp, synthetic construct
  misc_feature 1..20: note = Description of Artificial Sequence: Synthetic primer
  source 1..20: mol_type = other DNA
tggtcagtacaagcacatac

SEQ ID NO: 187 - DNA, 20 bp, synthetic construct
  misc_feature 1..20: note = Description of Artificial Sequence: Synthetic primer
  source 1..20: mol_type = other DNA
atgggctttcttgatgtaac

SEQ ID NO: 188 - DNA, 16 bp, synthetic construct
  misc_feature 1..16: note = Description of Artificial Sequence: Synthetic primer
  source 1..16: mol_type = other DNA
ggttccgccaagagat

SEQ ID NO: 189 - DNA, 21 bp, synthetic construct
  misc_feature 1..21: note = Description of Artificial Sequence: Synthetic primer
  source 1..21: mol_type = other DNA
ggccaatttcccattctaata

SEQ ID NO: 190 - DNA, 16 bp, synthetic construct
  misc_feature 1..16: note = Description of Artificial Sequence: Synthetic primer
  source 1..16: mol_type = other DNA
tgacaaaccgagcact

SEQ ID NO: 191 - DNA, 19 bp, synthetic construct
  misc_feature 1..19: note = Description of Artificial Sequence: Synthetic primer
  source 1..19: mol_type = other DNA
cttcatcccccagtaagtc

SEQ ID NO: 192 - DNA, 20 bp, synthetic construct
  misc_feature 1..20: note = Description of Artificial Sequence: Synthetic primer
  source 1..20: mol_type = other DNA
ttctgggagttttcgtatca

SEQ ID NO: 193 - DNA, 17 bp, synthetic construct
  misc_feature 1..17: note = Description of Artificial Sequence: Synthetic primer
  source 1..17: mol_type = other DNA
tccacagccacatcttt

SEQ ID NO: 194 - DNA, 17 bp, synthetic construct
  misc_feature 1..17: note = Description of Artificial Sequence: Synthetic primer
  source 1..17: mol_type = other DNA
ctgacagtgcgtacatc

SEQ ID NO: 195 - DNA, 21 bp, synthetic construct
  misc_feature 1..21: note = Description of Artificial Sequence: Synthetic primer
  source 1..21: mol_type = other DNA
tcattccaaagtcagctatct

SEQ ID NO: 196 - DNA, 19 bp, synthetic construct
  misc_feature 1..19: note = Description of Artificial Sequence: Synthetic primer
  source 1..19: mol_type = other DNA
aggtccacatccattcatc

SEQ ID NO: 197 - DNA, 17 bp, synthetic construct
  misc_feature 1..17: note = Description of Artificial Sequence: Synthetic primer
  source 1..17: mol_type = other DNA
cataggcatgggtgagt

SEQ ID NO: 198 - DNA, 21 bp, synthetic construct
  misc_feature 1..21: note = Description of Artificial Sequence: Synthetic primer
  source 1..21: mol_type = other DNA
ccttcagtccggttttatttg

SEQ ID NO: 199 - DNA, 19 bp, synthetic construct
  misc_feature 1..19: note = Description of Artificial Sequence: Synthetic primer
  source 1..19: mol_type = other DNA
cagaaagcggtgacttact

SEQ ID NO: 200 - DNA, 17 bp, synthetic construct
  misc_feature 1..17: note = Description of Artificial Sequence: Synthetic primer
  source 1..17: mol_type = other DNA
gctaatggcccgttctc

SEQ ID NO: 201 - DNA, 17 bp, synthetic construct
  misc_feature 1..17: note = Description of Artificial Sequence: Synthetic primer
  source 1..17: mol_type = other DNA
cccaccagaccatgaga

SEQ ID NO: 202 - DNA, 20 bp, synthetic construct
  misc_feature 1..20: note = Description of Artificial Sequence: Synthetic primer
  source 1..20: mol_type = other DNA
agccaatattgtctttgtgt

SEQ ID NO: 203 - DNA, 20 bp, synthetic construct
  misc_feature 1..20: note = Description of Artificial Sequence: Synthetic primer
  source 1..20: mol_type = other DNA
ctccttctgcatggtattct

SEQ ID NO: 204 - DNA, 22 bp, synthetic construct
  misc_feature 1..22: note = Description of Artificial Sequence: Synthetic primer
  source 1..22: mol_type = other DNA
cattagcatcaggattatgact

SEQ ID NO: 205 - DNA, 16 bp, synthetic construct
  misc_feature 1..16: note = Description of Artificial Sequence: Synthetic primer
  source 1..16: mol_type = other DNA
ccagagcccagacctg

SEQ ID NO: 206 - DNA, 23 bp, synthetic construct
  misc_feature 1..23: note = Description of Artificial Sequence: Synthetic primer
  source 1..23: mol_type = other DNA
ggagttactatatgggaactgat

SEQ ID NO: 207 - DNA, 22 bp, synthetic construct
  misc_feature 1..22: note = Description of Artificial Sequence: Synthetic primer
  source 1..22: mol_type = other DNA
aactctgagtcttgtttctaca

SEQ ID NO: 208 - DNA, 20 bp, synthetic construct
  misc_feature 1..20: note = Description of Artificial Sequence: Synthetic primer
  source 1..20: mol_type = other DNA
cctgcatgaatttcaatgac

SEQ ID NO: 209 - DNA, 20 bp, synthetic construct
  misc_feature 1..20: note = Description of Artificial Sequence: Synthetic primer
  source 1..20: mol_type = other DNA
gttatgcagacaccattcat

SEQ ID NO: 210 - DNA, 20 bp, synthetic construct
  misc_feature 1..20: note = Description of Artificial Sequence: Synthetic primer
  source 1..20: mol_type = other DNA
aattgcattcacacgttaac

SEQ ID NO: 211 - DNA, 23 bp, synthetic construct
  misc_feature 1..23: note = Description of Artificial Sequence: Synthetic primer
  source 1..23: mol_type = other DNA
ccttgactaaatctaccatgttt

SEQ ID NO: 212 - DNA, 21 bp, synthetic construct
  misc_feature 1..21: note = Description of Artificial Sequence: Synthetic primer
  source 1..21: mol_type = other DNA
ccagtgtctgagaacattagt

SEQ ID NO: 213 - DNA, 20 bp, synthetic construct
  misc_feature 1..20: note = Description of Artificial Sequence: Synthetic primer
  source 1..20: mol_type = other DNA
agacagcacagaattgatac

SEQ ID NO: 214 - DNA, 23 bp, synthetic construct
  misc_feature 1..23: note = Description of Artificial Sequence: Synthetic primer
  source 1..23: mol_type = other DNA
tcagtgtattcatcgagatttag

SEQ ID NO: 215 - DNA, 19 bp, synthetic construct
  misc_feature 1..19: note = Description of Artificial Sequence: Synthetic primer
  source 1..19: mol_type = other DNA
tgtctgcaaggtttacagt

SEQ ID NO: 216 - DNA, 16 bp, synthetic construct
  misc_feature 1..16: note = Description of Artificial Sequence: Synthetic primer
  source 1..16: mol_type = other DNA
gctgtgcgtcactgta

SEQ ID NO: 217 - DNA, 13 bp, synthetic construct
  misc_feature 1..13: note = Description of Artificial Sequence: Synthetic primer
  source 1..13: mol_type = other DNA
cgcaggcggcaga

SEQ ID NO: 218 - DNA, 14 bp, synthetic construct
  misc_feature 1..14: note = Description of Artificial Sequence: Synthetic primer
  source 1..14: mol_type = other DNA
ggaaggcggtgttg

SEQ ID NO: 219 - DNA, 14 bp, synthetic construct
  misc_feature 1..14: note = Description of Artificial Sequence: Synthetic primer
  source 1..14: mol_type = other DNA
gcctgctgtggccc

SEQ ID NO: 220 - DNA, 15 bp, synthetic construct
  misc_feature 1..15: note = Description of Artificial Sequence: Synthetic primer
  source 1..15: mol_type = other DNA
agggcgacgagaaac

SEQ ID NO: 221 - DNA, 22 bp, synthetic construct
  misc_feature 1..22: note = Description of Artificial Sequence: Synthetic primer
  source 1..22: mol_type = other DNA
tcctctagctatcttaatgact

SEQ ID NO: 222 - DNA, 20 bp, synthetic construct
  misc_feature 1..20: note = Description of Artificial Sequence: Synthetic primer
  source 1..20: mol_type = other DNA
gcttactggaagttgacttt

SEQ ID NO: 223 - DNA, 17 bp, synthetic construct
  misc_feature 1..17: note = Description of Artificial Sequence: Synthetic primer
  source 1..17: mol_type = other DNA
ggaagcaggtggtcatt

SEQ ID NO: 224 - DNA, 18 bp, synthetic construct
  misc_feature 1..18: note = Description of Artificial Sequence: Synthetic primer
  source 1..18: mol_type = other DNA
tggcttctcctctacaga

SEQ ID NO: 225 - DNA, 20 bp, synthetic construct
  misc_feature 1..20: note = Description of Artificial Sequence: Synthetic primer
  source 1..20: mol_type = other DNA
ggatgctgcagaagctataa

SEQ ID NO: 226 - DNA, 20 bp, synthetic construct
  misc_feature 1..20: note = Description of Artificial Sequence: Synthetic primer
  source 1..20: mol_type = other DNA
gttcaagctgaagaagatgt

SEQ ID NO: 227 - DNA, 18 bp, synthetic construct
  misc_feature 1..18: note = Description of Artificial Sequence: Synthetic primer
  source 1..18: mol_type = other DNA
gctcagttcctggacaaa

SEQ ID NO: 228 - DNA, 22 bp, synthetic construct
  misc_feature 1..22: note = Description of Artificial Sequence: Synthetic primer
  source 1..22: mol_type = other DNA
cctttgaatgcagaagattctt

SEQ ID NO: 229 - DNA, 18 bp, synthetic construct
  misc_feature 1..18: note = Description of Artificial Sequence: Synthetic primer
  source 1..18: mol_type = other DNA
agcagagaatgggtactc

SEQ ID NO: 230 - DNA, 18 bp, synthetic construct
  misc_feature 1..18: note = Description of Artificial Sequence: Synthetic primer
  source 1..18: mol_type = other DNA
gttgtctttggcaaggat

SEQ ID NO: 231 - DNA, 21 bp, synthetic construct
  misc_feature 1..21: note = Description of Artificial Sequence: Synthetic primer
  source 1..21: mol_type = other DNA
gcactgtaataatccagactg

SEQ ID NO: 232 - DNA, 17 bp, synthetic construct
  misc_feature 1..17: note = Description of Artificial Sequence: Synthetic primer
  source 1..17: mol_type = other DNA
gtgggagaccttgaaca

SEQ ID NO: 233 - DNA, 17 bp, synthetic construct
  misc_feature 1..17: note = Description of Artificial Sequence: Synthetic primer
  source 1..17: mol_type = other DNA
gccatggagtcgatgag

SEQ ID NO: 234 - DNA, 19 bp, synthetic construct
  misc_feature 1..19: note = Description of Artificial Sequence: Synthetic primer
  source 1..19: mol_type = other DNA
gcctgacaaatccagagta

SEQ ID NO: 235 - DNA, 19 bp, synthetic construct
  misc_feature 1..19: note = Description of Artificial Sequence: Synthetic primer
  source 1..19: mol_type = other DNA
tgatgaaccggtcctttac

SEQ ID NO: 236 - DNA, 21 bp, synthetic construct
  misc_feature 1..21: note = Description of Artificial Sequence: Synthetic primer
  source 1..21: mol_type = other DNA
cgacgacaatcttaaactgta

SEQ ID NO: 237 - DNA, 20 bp, synthetic construct
  misc_feature 1..20: note = Description of Artificial Sequence: Synthetic primer
  source 1..20: mol_type = other DNA
acaacccactgaggtatatg

SEQ ID NO: 238 - DNA, 19 bp, synthetic construct
  misc_feature 1..19: note = Description of Artificial Sequence: Synthetic primer
  source 1..19: mol_type = other DNA
tgtatggtaggaccaccag

SEQ ID NO: 239 - DNA, 20 bp, synthetic construct
  misc_feature 1..20: note = Description of Artificial Sequence: Synthetic primer
  source 1..20: mol_type = other DNA
aaacagattcctccttgtca

SEQ ID NO: 240 - DNA, 19 bp, synthetic construct
  misc_feature 1..19: note = Description of Artificial Sequence: Synthetic primer
  source 1..19: mol_type = other DNA
gcacctgttttgttgtgta

SEQ ID NO: 241 - DNA, 14 bp, synthetic construct
  misc_feature 1..14: note = Description of Artificial Sequence: Synthetic primer
  source 1..14: mol_type = other DNA
cccacccgtgaccg

SEQ ID NO: 242 - DNA, 16 bp, synthetic construct
  misc_feature 1..16: note = Description of Artificial Sequence: Synthetic primer
  source 1..16: mol_type = other DNA
caggtgcagccacaaa

SEQ ID NO: 243 - DNA, 20 bp, synthetic construct
  misc_feature 1..20: note = Description of Artificial Sequence: Synthetic primer
  source 1..20: mol_type = other DNA
tctacctggagattgacaac

SEQ ID NO: 244 - DNA, 16 bp, synthetic construct
  misc_feature 1..16: note = Description of Artificial Sequence: Synthetic primer
  source 1..16: mol_type = other DNA
caagcaccccatcaag

SEQ ID NO: 245 - DNA, 13 bp, synthetic construct
  misc_feature 1..13: note = Description of Artificial Sequence: Synthetic primer
  source 1..13: mol_type = other DNA
ccggcacgctggt

SEQ ID NO: 246 - DNA, 15 bp, synthetic construct
  misc_feature 1..15: note = Description of Artificial Sequence: Synthetic primer
  source 1..15: mol_type = other DNA
ccacggtggctacaa

SEQ ID NO: 247 - DNA, 20 bp, synthetic construct
  misc_feature 1..20: note = Description of Artificial Sequence: Synthetic primer
  source 1..20: mol_type = other DNA
acctgtttgttggacatact

SEQ ID NO: 248 - DNA, 19 bp, synthetic construct
  misc_feature 1..19: note = Description of Artificial Sequence: Synthetic primer
  source 1..19: mol_type = other DNA
aagactcggatgatgtacc

SEQ ID NO: 249 - DNA, 19 bp, synthetic construct
  misc_feature 1..19: note = Description of Artificial Sequence: Synthetic primer
  source 1..19: mol_type = other DNA
ggttaccccatggaactta

SEQ ID NO: 250 - DNA, 20 bp, synthetic construct
  misc_feature 1..20: note = Description of Artificial Sequence: Synthetic primer
  source 1..20: mol_type = other DNA
caggaagctatccctattct

SEQ ID NO: 251 - DNA, 17 bp, synthetic construct
  misc_feature 1..17: note = Description of Artificial Sequence: Synthetic primer
  source 1..17: mol_type = other DNA
gttaccccaacggctac

SEQ ID NO: 252 - DNA, 20 bp, synthetic construct
  misc_feature 1..20: note = Description of Artificial Sequence: Synthetic primer
  source 1..20: mol_type = other DNA
tgcagatggcatcattaatc

SEQ ID NO: 253 - DNA, 18 bp, synthetic construct
  misc_feature 1..18: note = Description of Artificial Sequence: Synthetic primer
  source 1..18: mol_type = other DNA
cacccagaaagcagacta

SEQ ID NO: 254 - DNA, 18 bp, synthetic construct
  misc_feature 1..18: note = Description of Artificial Sequence: Synthetic primer
  source 1..18: mol_type = other DNA
cgacacacacgacaatac

SEQ ID NO: 255 - DNA, 18 bp, synthetic construct
  misc_feature 1..18: note = Description of Artificial Sequence: Synthetic primer
  source 1..18: mol_type = other DNA
gtcacagccttcttcatg

SEQ ID NO: 256 - DNA, 15 bp, synthetic construct
  misc_feature 1..15: note = Description of Artificial Sequence: Synthetic primer
  source 1..15: mol_type = other DNA
cgcatggcctcttct

SEQ ID NO: 257 - DNA, 16 bp, synthetic construct
  misc_feature 1..16: note = Description of Artificial Sequence: Synthetic primer
  source 1..16: mol_type = other DNA
gcaccgagacgatgaa

SEQ ID NO: 258 - DNA, 15 bp, synthetic construct
  misc_feature 1..15: note = Description of Artificial Sequence: Synthetic primer
  source 1..15: mol_type = other DNA
gcacctggctcctct

SEQ ID NO: 259 - DNA, 20 bp, synthetic construct
  misc_feature 1..20: note = Description of Artificial Sequence: Synthetic primer
  source 1..20: mol_type = other DNA
ccccatacaatttgatgaca

SEQ ID NO: 260 - DNA, 14 bp, synthetic construct
  misc_feature 1..14: note = Description of Artificial Sequence: Synthetic primer
  source 1..14: mol_type = other DNA
tccgccgcacttac

SEQ ID NO: 261 - DNA, 18 bp, synthetic construct
  misc_feature 1..18: note = Description of Artificial Sequence: Synthetic primer
  source 1..18: mol_type = other DNA
gtgagcaggtggaagtag

SEQ ID NO: 262 - DNA, 15 bp, synthetic construct
  misc_feature 1..15: note = Description of Artificial Sequence: Synthetic primer
  source 1..15: mol_type = other DNA
ccagatgagcagcgt

SEQ ID NO: 263 - DNA, 20 bp, synthetic construct
  misc_feature 1..20: note = Description of Artificial Sequence: Synthetic primer
  source 1..20: mol_type = other DNA
tcttcctcctcttcttcttc

SEQ ID NO: 264 - DNA, 16 bp, synthetic construct
  misc_feature 1..16: note = Description of Artificial Sequence: Synthetic primer
  source 1..16: mol_type = other DNA
cagcaagtgcccagta

SEQ ID NO: 265 - DNA, 16 bp, synthetic construct
  misc_feature 1..16: note = Description of Artificial Sequence: Synthetic primer
  source 1..16: mol_type = other DNA
ccgagtccagcacctc

SEQ ID NO: 266 - DNA, 16 bp, synthetic construct
  misc_feature 1..16: note = Description of Artificial Sequence: Synthetic primer
  source 1..16: mol_type = other DNA
aggctcccacctttca

SEQ ID NO: 267 - DNA, 18 bp, synthetic construct
  misc_feature 1..18: note = Description of Artificial Sequence: Synthetic primer
  source 1..18: mol_type = other DNA
acagaccctctcactcat

SEQ ID NO: 268 - DNA, 17 bp, synthetic construct
  misc_feature 1..17: note = Description of Artificial Sequence: Synthetic primer
  source 1..17: mol_type = other DNA
ccaagggtgcagttatg

SEQ ID NO: 269 - DNA, 17 bp, synthetic construct
  misc_feature 1..17: note = Description of Artificial Sequence: Synthetic primer
  source 1..17: mol_type = other DNA
tgcctcttgcttctctt

SEQ ID NO: 270 - DNA, 20 bp, synthetic construct
  misc_feature 1..20: note = Description of Artificial Sequence: Synthetic primer
  source 1..20: mol_type = other DNA
cctcactgattgctcttagg

SEQ ID NO: 271 - DNA, 16 bp, synthetic construct
  misc_feature 1..16: note = Description of Artificial Sequence: Synthetic primer
  source 1..16: mol_type = other DNA
gcagctgtgggttgat

SEQ ID NO: 272 - DNA, 16 bp, synthetic construct
  misc_feature 1..16: note = Description of Artificial Sequence: Synthetic primer
  source 1..16: mol_type = other DNA
ggcccctgtcatcttc

SEQ ID NO: 273 - DNA, 18 bp, synthetic construct
  misc_feature 1..18: note = Description of Artificial Sequence: Synthetic primer
  source 1..18: mol_type = other DNA
gtcctctgactgctcttt

SEQ ID NO: 274 - DNA, 17 bp, synthetic construct
  misc_feature 1..17: note = Description of Artificial Sequence: Synthetic primer
  source 1..17: mol_type = other DNA
gctggatccccactttt

SEQ ID NO: 275 - DNA, 17 bp, synthetic construct
  misc_feature 1..17: note = Description of Artificial Sequence: Synthetic primer
  source 1..17: mol_type = other DNA
tcacgttggtccacatc

SEQ ID NO: 276 - DNA, 18 bp, synthetic construct
  misc_feature 1..18: note = Description of Artificial Sequence: Synthetic primer
  source 1..18: mol_type = other DNA
acaggatgacaggaagag

SEQ ID NO: 277 - DNA, 20 bp, synthetic construct
  misc_feature 1..20: note = Description of Artificial Sequence: Synthetic primer
  source 1..20: mol_type = other DNA
acgatttcccttggagatat

SEQ ID NO: 278 - DNA, 20 bp, synthetic construct
  misc_feature 1..20: note = Description of Artificial Sequence: Synthetic primer
  source 1..20: mol_type = other DNA
agacaactgttcaaactgat

SEQ ID NO: 279 - DNA, 20 bp, synthetic construct
  misc_feature 1..20: note = Description of Artificial Sequence: Synthetic primer
  source 1..20: mol_type = other DNA
gaccccaagctttagtaaat

SEQ ID NO: 280 - DNA, 19 bp, synthetic construct
  misc_feature 1..19: note = Description of Artificial Sequence: Synthetic primer
  source 1..19: mol_type = other DNA
acaccctccattttatcac

SEQ ID NO: 281 - DNA, 20 bp, synthetic construct
  misc_feature 1..20: note = Description of Artificial Sequence: Synthetic primer
  source 1..20: mol_type = other DNA
cacgaatgtgtggttaactc

SEQ ID NO: 282 - DNA, 17 bp, synthetic construct
  misc_feature 1..17: note = Description of Artificial Sequence: Synthetic primer
  source 1..17: mol_type = other DNA
tttccttcccccttgtc

SEQ ID NO: 283 - DNA, 20 bp, synthetic construct
  misc_feature 1..20: note = Description of Artificial Sequence: Synthetic primer
  source 1..20: mol_type = other DNA
ttgtattctctgccttctct

SEQ ID NO: 284 - DNA, 18 bp, synthetic construct
  misc_feature 1..18: note = Description of Artificial Sequence: Synthetic primer
  source 1..18: mol_type = other DNA
aataaccgctcctcatca

SEQ ID NO: 285 - DNA, 22 bp, synthetic construct
  misc_feature 1..22: note = Description of Artificial Sequence: Synthetic primer
  source 1..22: mol_type = other DNA
ctgagactagatgacttttgtc

SEQ ID NO: 286 - DNA, 23 bp, synthetic construct
  misc_feature 1..23: note = Description of Artificial Sequence: Synthetic primer
  source 1..23: mol_type = other DNA
ctttacttaaatagggcaagttc

SEQ ID NO: 287 - DNA, 23 bp, synthetic construct
  misc_feature 1..23: note = Description of Artificial Sequence: Synthetic primer
  source 1..23: mol_type = other DNA
ttcctttatttttgttcccaaag

SEQ ID NO: 288 - DNA, 15 bp, synthetic construct
  misc_feature 1..15: note = Description of Artificial Sequence: Synthetic primer
  source 1..15: mol_type = other DNA
caacgccacaaccac

SEQ ID NO: 289 - DNA, 19 bp, synthetic construct
  misc_feature 1..19: note = Description of Artificial Sequence: Synthetic primer
  source 1..19: mol_type = other DNA
gtaccagatggatgtgaac

SEQ ID NO: 290 - DNA, 20 bp, synthetic construct
  misc_feature 1..20: note = Description of Artificial Sequence: Synthetic primer
  source 1..20: mol_type = other DNA
agagacatgcatgaacattt

SEQ ID NO: 291 - DNA, 19 bp, synthetic construct
  misc_feature 1..19: note = Description of Artificial Sequence: Synthetic primer
  source 1..19: mol_type = other DNA
cttgtctctgtgttcttgt

SEQ ID NO: 292 - DNA, 20 bp, synthetic construct
  misc_feature 1..20: note = Description of Artificial Sequence: Synthetic primer
  source 1..20: mol_type = other DNA
agttaacgtcttccttctct

SEQ ID NO: 293 - DNA, 15 bp, synthetic construct
  misc_feature 1..15: note = Description of Artificial Sequence: Synthetic primer
  source 1..15: mol_type = other DNA
gcatctgcctcacct

SEQ ID NO: 294 - DNA, 16 bp, synthetic construct
  misc_feature 1..16: note = Description of Artificial Sequence: Synthetic primer
  source 1..16: mol_type = other DNA
agccaggaacgtactg

SEQ ID NO: 295 - DNA, 20 bp, synthetic construct
  misc_feature 1..20: note = Description of Artificial Sequence: Synthetic primer
  source 1..20: mol_type = other DNA
aagggattgtgattgttcat

SEQ ID NO: 296 - DNA, 20 bp, synthetic construct
  misc_feature 1..20: note = Description of Artificial Sequence: Synthetic primer
  source 1..20: mol_type = other DNA
cctgatctccttagacaact

SEQ ID NO: 297 - DNA, 17 bp, synthetic construct
  misc_feature 1..17: note = Description of Artificial Sequence: Synthetic primer
  source 1..17: mol_type = other DNA
ataccctctcagcgtac

SEQ ID NO: 298 - DNA, 16 bp, synthetic construct
  misc_feature 1..16: note = Description of Artificial Sequence: Synthetic primer
  source 1..16: mol_type = other DNA
ggggatgagctacctg

SEQ ID NO: 299 - DNA, 16 bp, synthetic construct
  misc_feature 1..16: note = Description of Artificial Sequence: Synthetic primer
  source 1..16: mol_type = other DNA
ttggccagcaagaatg

SEQ ID NO: 300 - DNA, 18 bp, synthetic construct
  misc_feature 1..18: note = Description of Artificial Sequence: Synthetic primer
  source 1..18: mol_type = other DNA
cagtgcaaggtttacaca

SEQ ID NO: 301 - DNA, 21 bp, synthetic construct
  misc_feature 1..21: note = Description of Artificial Sequence: Synthetic primer
  source 1..21: mol_type = other DNA
gaaaggagagcaggataataa

SEQ ID NO: 302 - DNA, 24 bp, synthetic construct
  misc_feature 1..24: note = Description of Artificial Sequence: Synthetic primer
  source 1..24: mol_type = other DNA
cactgatatttaaatgccttagag

SEQ ID NO: 303 - DNA, 18 bp, synthetic construct
  misc_feature 1..18: note = Description of Artificial Sequence: Synthetic primer
  source 1..18: mol_type = other DNA
cagcagcttggtttcttc

SEQ ID NO: 304 - DNA, 17 bp, synthetic construct
  misc_feature 1..17: note = Description of Artificial Sequence: Synthetic primer
  source 1..17: mol_type = other DNA
tgcaacgtgtgtagaca

SEQ ID NO: 305 - DNA, 17 bp, synthetic construct
  misc_feature 1..17: note = Description of Artificial Sequence: Synthetic primer
  source 1..17: mol_type = other DNA
tcccaaccatgacaaga

SEQ ID NO: 306 - DNA, 21 bp, synthetic construct
  misc_feature 1..21: note = Description of Artificial Sequence: Synthetic primer
  source 1..21: mol_type = other DNA
gctacttgcaatgatatacac

SEQ ID NO: 307 - DNA, 22 bp, synthetic construct
  misc_feature 1..22: note = Description of Artificial Sequence: Synthetic primer
  source 1..22: mol_type = other DNA
cacccaatgaagaatgtaattg

SEQ ID NO: 308 - DNA, 17 bp, synthetic construct
  misc_feature 1..17: note = Description of Artificial Sequence: Synthetic primer
  source 1..17: mol_type = other DNA
agcccagccatttctaa

SEQ ID NO: 309 - DNA, 16 bp, synthetic construct
  misc_feature 1..16: note = Description of Artificial Sequence: Synthetic primer
  source 1..16: mol_type = other DNA
ctggctgctgaagtct

SEQ ID NO: 310 - DNA, 17 bp, synthetic construct
  misc_feature 1..17: note = Description of Artificial Sequence: Synthetic primer
  source 1..17: mol_type = other DNA
cactgtggaggcatttg

SEQ ID NO: 311 - DNA, 15 bp, synthetic construct
  misc_feature 1..15: note = Description of Artificial Sequence: Synthetic primer
  source 1..15: mol_type = other DNA
cagtggctcaagcac

SEQ ID NO: 312 - DNA, 14 bp, synthetic construct
  misc_feature 1..14: note = Description of Artificial Sequence: Synthetic primer
  source 1..14: mol_type = other DNA
gaggagcccgtgtc

SEQ ID NO: 313 - DNA, 15 bp, synthetic construct
  misc_feature 1..15: note = Description of Artificial Sequence: Synthetic primer
  source 1..15: mol_type = other DNA
ctgcagctggtcctt

SEQ ID NO: 314 - DNA, 16 bp, synthetic construct
  misc_feature 1..16: note = Description of Artificial Sequence: Synthetic primer
  source 1..16: mol_type = other DNA
gcaggagctgacagta

SEQ ID NO: 315 - DNA, 17 bp, synthetic construct
  misc_feature 1..17: note = Description of Artificial Sequence: Synthetic primer
  source 1..17: mol_type = other DNA
cggtagttgcccttctc

SEQ ID NO: 316 - DNA, 16 bp, synthetic construct
  misc_feature 1..16: note = Description of Artificial Sequence: Synthetic primer
  source 1..16: mol_type = other DNA
cgctgtgtcctttcag

SEQ ID NO: 317 - DNA, 22 bp, synthetic construct
  misc_feature 1..22: note = Description of Artificial Sequence: Synthetic primer
  source 1..22: mol_type = other DNA
gacattttcaaagcagtgtatc

SEQ ID NO: 318 - DNA, 18 bp, synthetic construct
  misc_feature 1..18: note = Description of Artificial Sequence: Synthetic primer
  source 1..18: mol_type = other DNA
ccagtccctctggaataa

SEQ ID NO: 319 - DNA, 19 bp, synthetic construct
  misc_feature 1..19: note = Description of Artificial Sequence: Synthetic primer
  source 1..19: mol_type = other DNA
ctctatagtggggtcgtat

SEQ ID NO: 320 - DNA, 20 bp, synthetic construct
  misc_feature 1..20: note = Description of Artificial Sequence: Synthetic primer
  source 1..20: mol_type = other DNA
acattattgccaacatgact

SEQ ID NO: 321 - DNA, 20 bp, synthetic construct
  misc_feature 1..20: note = Description of Artificial Sequence: Synthetic primer
  source 1..20: mol_type = other DNA
catactcaacacgattctgt

SEQ ID NO: 322 - DNA, 17 bp, synthetic construct
  misc_feature 1..17: note = Description of Artificial Sequence: Synthetic primer
  source 1..17: mol_type = other DNA
ggcacggttgaatgtaa

SEQ ID NO: 323 - DNA, 21 bp, synthetic construct
  misc_feature 1..21: note = Description of Artificial Sequence: Synthetic primer
  source 1..21: mol_type = other DNA
ccacatttctcttccattgta

SEQ ID NO: 324 - DNA, 29 bp, synthetic construct
  misc_feature 1..29: note = Description of Artificial Sequence: Synthetic primer
  source 1..29: mol_type = other DNA
agacaataattattaaaaggtgatctatt

SEQ ID NO: 325 - DNA, 16 bp, synthetic construct
  misc_feature 1..16: note = Description of Artificial Sequence: Synthetic primer
  source 1..16: mol_type = other DNA
ttagcgagtgcccatt

SEQ ID NO: 326 - DNA, 18 bp, synthetic construct
  misc_feature 1..18: note = Description of Artificial Sequence: Synthetic primer
  source 1..18: mol_type = other DNA
tgtcccacttgattcagt

SEQ ID NO: 327 - DNA, 18 bp, synthetic construct
  misc_feature 1..18: note = Description of Artificial Sequence: Synthetic primer
  source 1..18: mol_type = other DNA
cgtgagtacccattctct

SEQ ID NO: 328 - DNA, 22 bp, synthetic construct
  misc_feature 1..22: note = Description of Artificial Sequence: Synthetic primer
  source 1..22: mol_type = other DNA
ccaaagacaacttcattagact

SEQ ID NO: 329 - DNA, 26 bp, synthetic construct
  misc_feature 1..26: note = Description of Artificial Sequence: Synthetic primer
  source 1..26: mol_type = other DNA
gtatttatttcagtgttacttacctg

SEQ ID NO: 330 - DNA, 20 bp, synthetic construct
  misc_feature 1..20: note = Description of Artificial Sequence: Synthetic primer
  source 1..20: mol_type = other DNA
ggatcatattcgtccacaaa

SEQ ID NO: 331 - DNA, 21 bp, synthetic construct
  misc_feature 1..21: note = Description of Artificial Sequence: Synthetic primer
  source 1..21: mol_type = other DNA
ctttctccagctaattcatct

SEQ ID NO: 332 - DNA, 17 bp, synthetic construct
  misc_feature 1..17: note = Description of Artificial Sequence: Synthetic primer
  source 1..17: mol_type = other DNA
ctgcagccagaaagact

SEQ ID NO: 333 - DNA, 19 bp, synthetic construct
  misc_feature 1..19: note = Description of Artificial Sequence: Synthetic primer
  source 1..19: mol_type = other DNA
tcctctcgtttccttacat

SEQ ID NO: 334 - DNA, 18 bp, synthetic construct
  misc_feature 1..18: note = Description of Artificial Sequence: Synthetic primer
  source 1..18: mol_type = other DNA
caaagcaagccagattct

SEQ ID NO: 335 - DNA, 17 bp, synthetic construct
  misc_feature 1..17: note = Description of Artificial Sequence: Synthetic primer
  source 1..17: mol_type = other DNA
gcactgggtcaaagtct

SEQ ID NO: 336 - DNA, 19 bp, synthetic construct
  misc_feature 1..19: note = Description of Artificial Sequence: Synthetic primer
  source 1..19: mol_type = other DNA
cagtgctaaccaagttctt

SEQ ID NO: 337 - DNA, 15 bp, synthetic construct
  misc_feature 1..15: note = Description of Artificial Sequence: Synthetic primer
  source 1..15: mol_type = other DNA
cgctcctgggaatct

SEQ ID NO: 338 - DNA, 18 bp, synthetic construct
  misc_feature 1..18: note = Description of Artificial Sequence: Synthetic primer
  source 1..18: mol_type = other DNA
cagtcaaggttgctgatt

SEQ ID NO: 339 - DNA, 14 bp, synthetic construct
  misc_feature 1..14: note = Description of Artificial Sequence: Synthetic primer
  source 1..14: mol_type = other DNA
ggcgtcaggaactg

SEQ ID NO: 340 - DNA, 16 bp, synthetic construct
  misc_feature 1..16: note = Description of Artificial Sequence: Synthetic primer
  source 1..16: mol_type = other DNA
cggcctcgatcttgta

SEQ ID NO: 341 - DNA, 14 bp, synthetic construct
  misc_feature 1..14: note = Description of Artificial Sequence: Synthetic primer
  source 1..14: mol_type = other DNA
cagctcctcctcgc

SEQ ID NO: 342 - DNA, 21 bp, synthetic construct
  misc_feature 1..21: note = Description of Artificial Sequence: Synthetic primer
  source 1..21: mol_type = other DNA
ggtgggatcatattcatctac

SEQ ID NO: 343 - DNA, 22 bp, synthetic construct
  misc_feature 1..22: note = Description of Artificial Sequence: Synthetic primer
  source 1..22: mol_type = other DNA
gtctgaactgaagataatgact

SEQ ID NO: 344 - DNA, 16 bp, synthetic construct
  misc_feature 1..16: note = Description of Artificial Sequence: Synthetic primer
  source 1..16: mol_type = other DNA
tgtccaccgtgatctg

SEQ ID NO: 345 - DNA, 19 bp, synthetic construct
  misc_feature 1..19: note = Description of Artificial Sequence: Synthetic primer
  source 1..19: mol_type = other DNA
tcgtctgggaactatactc

SEQ ID NO: 346 - DNA, 18 bp, synthetic construct
  misc_feature 1..18: note = Description of Artificial Sequence: Synthetic primer
  source 1..18: mol_type = other DNA
tgtactgctcccagaaga

SEQ ID NO: 347 - DNA, 17 bp, synthetic construct
  misc_feature 1..17: note = Description of Artificial Sequence: Synthetic primer
  source 1..17: mol_type = other DNA
tgcaccaggagtttgta

SEQ ID NO: 348 - DNA, 15 bp, synthetic construct
  misc_feature 1..15: note = Description of Artificial Sequence: Synthetic primer
  source 1..15: mol_type = other DNA
gagggtgtcctgtgt

SEQ ID NO: 349 - DNA, 17 bp, synthetic construct
  misc_feature 1..17: note = Description of Artificial Sequence: Synthetic primer
  source 1..17: mol_type = other DNA
gccacagcagtctgaaa

SEQ ID NO: 350 - DNA, 19 bp, synthetic construct
  misc_feature 1..19: note = Description of Artificial Sequence: Synthetic primer
  source 1..19: mol_type = other DNA
aggttcgctgcttttaatc

SEQ ID NO: 351 - DNA, 16 bp, synthetic construct
  misc_feature 1..16: note = Description of Artificial Sequence: Synthetic primer
  source 1..16: mol_type = other DNA
cccgggggattaaagc

SEQ ID NO: 352 - DNA, 18 bp, synthetic construct
  misc_feature 1..18: note = Description of Artificial Sequence: Synthetic primer
  source 1..18: mol_type = other DNA
ggtcagctactcctcttc

SEQ ID NO: 353 - DNA, 17 bp, synthetic construct
  misc_feature 1..17: note = Description of Artificial Sequence: Synthetic primer
  source 1..17: mol_type = other DNA
cccctccttcctagaga

SEQ ID NO: 354 - DNA, 18 bp, synthetic construct
  misc_feature 1..18: note = Description of Artificial Sequence: Synthetic primer
  source 1..18: mol_type = other DNA
gtgctgcatttcagagaa

SEQ ID NO: 355 - DNA, 19 bp, synthetic construct
  misc_feature 1..19: note = Description of Artificial Sequence: Synthetic primer
  source 1..19: mol_type = other DNA
gtgcagaacatcaagttca

SEQ ID NO: 356 - DNA, 18 bp, synthetic construct
  misc_feature 1..18: note = Description of Artificial Sequence: Synthetic primer
  source 1..18: mol_type = other DNA
tggctttgtgctcattac

SEQ ID NO: 357 - DNA, 17 bp, synthetic construct
  misc_feature 1..17: note = Description of Artificial Sequence: Synthetic primer
  source 1..17: mol_type = other DNA
ctgctctcaggttgact

SEQ ID NO: 358 - DNA, 15 bp, synthetic construct
  misc_feature 1..15: note = Description of Artificial Sequence: Synthetic primer
  source 1..15: mol_type = other DNA
gagctggggactctt

SEQ ID NO: 359 - DNA, 19 bp, synthetic construct
  misc_feature 1..19: note = Description of Artificial Sequence: Synthetic primer
  source 1..19: mol_type = other DNA
caggagtcatgactctgtt

SEQ ID NO: 360 - DNA, 17 bp, synthetic construct
  misc_feature 1..17: note = Description of Artificial Sequence: Synthetic primer
  source 1..17: mol_type = other DNA
tggcctttgacctcaat

SEQ ID NO: 361 - DNA, 14 bp, synthetic construct
  misc_feature 1..14: note = Description of Artificial Sequence: Synthetic primer
  source 1..14: mol_type = other DNA
gcccgcaggtactt

SEQ ID NO: 362 - DNA, 15 bp, synthetic construct
  misc_feature 1..15: note = Description of Artificial Sequence: Synthetic primer
  source 1..15: mol_type = other DNA
atcctccggctgaag

SEQ ID NO: 363 - DNA, 15 bp, synthetic construct
  misc_feature 1..15: note = Description of Artificial Sequence: Synthetic primer
  source 1..15: mol_type = other DNA
ctggagtgagccctg

SEQ ID NO: 364 - DNA, 17 bp, synthetic construct
  misc_feature 1..17: note = Description of Artificial Sequence: Synthetic primer
  source 1..17: mol_type = other DNA
gcagtgctaggaaagag

SEQ ID NO: 365 - DNA, 13 bp, synthetic construct
  misc_feature 1..13: note = Description of Artificial Sequence: Synthetic primer
  source 1..13: mol_type = other DNA
tgcagggtggcaa

SEQ ID NO: 366 - DNA, 16 bp, synthetic construct
  misc_feature 1..16: note = Description of Artificial Sequence: Synthetic primer
  source 1..16: mol_type = other DNA
cgtcatgtgctgtgac

SEQ ID NO: 367 - DNA, 21 bp, synthetic construct
  misc_feature 1..21: note = Description of Artificial Sequence: Synthetic primer
  source 1..21: mol_type = other DNA
gtgtttctgtcatccaaatac

SEQ ID NO: 368 - DNA, 17 bp, synthetic construct
  misc_feature 1..17: note = Description of Artificial Sequence: Synthetic primer
  source 1..17: mol_type = other DNA
tgccctggtaggttttc

SEQ ID NO: 369 - DNA, 17 bp, synthetic construct
  misc_feature 1..17: note = Description of Artificial Sequence: Synthetic primer
  source 1..17: mol_type = other DNA
caagggggactgtagat

SEQ ID NO: 370 - DNA, 17 bp, synthetic construct
  misc_feature 1..17: note = Description of Artificial Sequence: Synthetic primer
  source 1..17: mol_type = other DNA
ggtctgacgggtagagt

SEQ ID NO: 371 - DNA, 17 bp, synthetic construct
  misc_feature 1..17: note = Description of Artificial Sequence: Synthetic primer
  source 1..17: mol_type = other DNA
tctgtctccccacagag

SEQ ID NO: 372 - DNA, 18 bp, synthetic construct
  misc_feature 1..18: note = Description of Artificial Sequence: Synthetic primer
  source 1..18: mol_type = other DNA
tgaagtgtgctctgaaca

SEQ ID NO: 373 - DNA, 18 bp, synthetic construct
  misc_feature 1..18: note = Description of Artificial Sequence: Synthetic primer
  source 1..18: mol_type = other DNA
atgcttgctctgatagga

SEQ ID NO: 374 - DNA, 23 bp, synthetic construct
  misc_feature 1..23: note = Description of Artificial Sequence: Synthetic primer
  source 1..23: mol_type = other DNA
acacaagactcagaatagataca

SEQ ID NO: 375 - DNA, 20 bp, synthetic construct
  misc_feature 1..20: note = Description of Artificial Sequence: Synthetic primer
  source 1..20: mol_type = other DNA
atgtctcttcttcctacctg

SEQ ID NO: 376 - DNA, 17 bp, synthetic construct
  misc_feature 1..17: note = Description of Artificial Sequence: Synthetic primer
  source 1..17: mol_type = other DNA
gccacacgtggtattca

SEQ ID NO: 377 - DNA, 18 bp, synthetic construct
  misc_feature 1..18: note = Description of Artificial Sequence: Synthetic primer
  source 1..18: mol_type = other DNA
tgagctccctacctgatt

SEQ ID NO: 378 - DNA, 19 bp, synthetic construct
  misc_feature 1..19: note = Description of Artificial Sequence: Synthetic primer
  source 1..19: mol_type = other DNA
caccttctccagcattttc

SEQ ID NO: 379 - DNA, 19 bp, synthetic construct
  misc_feature 1..19: note = Description of Artificial Sequence: Synthetic primer
  source 1..19: mol_type = other DNA
catcatcctcacctgactc

SEQ ID NO: 380 - DNA, 21 bp, synthetic construct
  misc_feature 1..21: note = Description of Artificial Sequence: Synthetic primer
  source 1..21: mol_type = other DNA
ttcaaaatgtagaccacagac

SEQ ID NO: 381 - DNA, 21 bp, synthetic construct
  misc_feature 1..21: note = Description of Artificial Sequence: Synthetic primer
  source 1..21: mol_type = other DNA
cggaagaactctccagtattc

SEQ ID NO: 382 - DNA, 19 bp, synthetic construct
  misc_feature 1..19: note = Description of Artificial Sequence: Synthetic primer
  source 1..19: mol_type = other DNA
ccttgttgaaggagcagaa

SEQ ID NO: 383 - DNA, 15 bp, synthetic construct
  misc_feature 1..15: note = Description of Artificial Sequence: Synthetic primer
  source 1..15: mol_type = other DNA
ccagagcccgactcg

SEQ ID NO: 384 - DNA, 19 bp, synthetic construct
  misc_feature 1..19: note = Description of Artificial Sequence: Synthetic primer
  source 1..19: mol_type = other DNA
tctccaagatgggatactc

SEQ ID NO: 385 - DNA, 16 bp, synthetic construct
  misc_feature 1..16: note = Description of Artificial Sequence: Synthetic primer
  source 1..16: mol_type = other DNA
ggcgtctgcgtacttc

SEQ ID NO: 386 - DNA, 20 bp, synthetic construct
  misc_feature 1..20: note = Description of Artificial Sequence: Synthetic primer
  source 1..20: mol_type = other DNA
cagggaccttaccttataca

SEQ ID NO: 387 - DNA, 15 bp, synthetic construct
  misc_feature 1..15: note = Description of Artificial Sequence: Synthetic primer
  source 1..15: mol_type = other DNA
cccccacacagcaaa

SEQ ID NO: 388 - DNA, 21 bp, synthetic construct
  misc_feature 1..21: note = Description of Artificial Sequence: Synthetic primer
  source 1..21: mol_type = other DNA
gtatctcccttccctgattac

SEQ ID NO: 389 - DNA, 15 bp, synthetic construct
  misc_feature 1..15: note = Description of Artificial Sequence: Synthetic primer
  source 1..15: mol_type = other DNA
tggtccctggtgtca

SEQ ID NO: 390 - DNA, 17 bp, synthetic construct
  misc_feature 1..17: note = Description of Artificial Sequence: Synthetic primer
  source 1..17: mol_type = other DNA
aggcgttctcctttctc

SEQ ID NO: 391 - DNA, 18 bp, synthetic construct
  misc_feature 1..18: note = Description of Artificial Sequence: Synthetic primer
  source 1..18: mol_type = other DNA
gcagtgagtgggtacctc

SEQ ID NO: 392 - DNA, 18 bp, synthetic construct
  misc_feature 1..18: note = Description of Artificial Sequence: Synthetic primer
  source 1..18: mol_type = other DNA
ccggacatggtctaagag

SEQ ID NO: 393 - DNA, 18 bp, synthetic construct
  misc_feature 1..18: note = Description of Artificial Sequence: Synthetic primer
  source 1..18: mol_type = other DNA
ccatctgcatggtactct

SEQ ID NO: 394 - DNA, 21 bp, synthetic construct
  misc_feature 1..21: note = Description of Artificial Sequence: Synthetic primer
  source 1..21: mol_type = other DNA
gtgctctcattttaaagatgg

SEQ ID NO: 395 - DNA, 21 bp, synthetic construct
  misc_feature 1..21: note = Description of Artificial Sequence: Synthetic primer
  source 1..21: mol_type = other DNA
gcttgtttgctgaatgttaac

SEQ ID NO: 396 - DNA, 18 bp, synthetic construct
  misc_feature 1..18: note = Description of Artificial Sequence: Synthetic primer
  source 1..18: mol_type = other DNA
gtgtgcagaacaatgtga

SEQ ID NO: 397 - DNA, 21 bp, synthetic construct
  misc_feature 1..21: note = Description of Artificial Sequence: Synthetic primer
  source 1..21: mol_type = other DNA
ggacttcaagaacttggatta

SEQ ID NO: 398 - DNA, 20 bp, synthetic construct
  misc_feature 1..20: note = Description of Artificial Sequence: Synthetic primer
  source 1..20: mol_type = other DNA
actatgggacttgaaaacgg

SEQ ID NO: 399 - DNA, 18 bp, synthetic construct
  misc_feature 1..18: note = Description of Artificial Sequence: Synthetic primer
  source 1..18: mol_type = other DNA
acaggccagtgtttacat

SEQ ID NO: 400 - DNA, 23 bp, synthetic construct
  misc_feature 1..23: note = Description of Artificial Sequence: Synthetic primer
  source 1..23: mol_type = other DNA
aacatcatcattagtggatctac

SEQ ID NO: 401 - DNA, 20 bp, synthetic construct
  misc_feature 1..20: note = Description of Artificial Sequence: Synthetic primer
  source 1..20: mol_type = other DNA
tgtgatcacatgcttacagt

SEQ ID NO: 402 - DNA, 22 bp, synthetic construct
  misc_feature 1..22: note = Description of Artificial Sequence: Synthetic primer
  source 1..22: mol_type = other DNA
gagaaattgcttgctttagatg

SEQ ID NO: 403 - DNA, 20 bp, synthetic construct
  misc_feature 1..20: note = Description of Artificial Sequence: Synthetic primer
  source 1..20: mol_type = other DNA
gtgtcagagatggagatgat

SEQ ID NO: 404 - DNA, 15 bp, synthetic construct
  misc_feature 1..15: note = Description of Artificial Sequence: Synthetic primer
  source 1..15: mol_type = other DNA
agcgcctggaagaga

SEQ ID NO: 405 - DNA, 17 bp, synthetic construct
  misc_feature 1..17: note = Description of Artificial Sequence: Synthetic primer
  source 1..17: mol_type = other DNA
ggcatgaggtcactgac

SEQ ID NO: 406 - DNA, 16 bp, synthetic construct
  misc_feature 1..16: note = Description of Artificial Sequence: Synthetic primer
  source 1..16: mol_type = other DNA
gctccaacccctagac

SEQ ID NO: 407 - DNA, 17 bp, synthetic construct
  misc_feature 1..17: note = Description of Artificial Sequence: Synthetic primer
  source 1..17: mol_type = other DNA
acaccaggtccttgaag

SEQ ID NO: 408 - DNA, 16 bp, synthetic construct
  misc_feature 1..16: note = Description of Artificial Sequence: Synthetic primer
  source 1..16: mol_type = other DNA
gggatgccactcacag

SEQ ID NO: 409 - DNA, 18 bp, synthetic construct
  misc_feature 1..18: note = Description of Artificial Sequence: Synthetic primer
  source 1..18: mol_type = other DNA
ggaagctggcaatctcta

SEQ ID NO: 410 - DNA, 21 bp, synthetic construct
  misc_feature 1..21: note = Description of Artificial Sequence: Synthetic primer
  source 1..21: mol_type = other DNA
cccgttctacgagaagaataa

SEQ ID NO: 411 - DNA, 14 bp, synthetic construct
  misc_feature 1..14: note = Description of Artificial Sequence: Synthetic primer
  source 1..14: mol_type = other DNA
gcccacctcgttgt

SEQ ID NO: 412 - DNA, 21 bp, synthetic construct
  misc_feature 1..21: note = Description of Artificial Sequence: Synthetic primer
  source 1..21: mol_type = other DNA
ccctaagtttgtaagtagtgc

SEQ ID NO: 413 - DNA, 20 bp, synthetic construct
  misc_feature 1..20: note = Description of Artificial Sequence: Synthetic primer
  source 1..20: mol_type = other DNA
agaagcaaagcgttctttac

SEQ ID NO: 414 - DNA, 17 bp, synthetic construct
  misc_feature 1..17: note = Description of Artificial Sequence: Synthetic primer
  source 1..17: mol_type = other DNA
agaccctgtaggaggac

SEQ ID NO: 415 - DNA, 20 bp, synthetic construct
  misc_feature 1..20: note = Description of Artificial Sequence: Synthetic primer
  source 1..20: mol_type = other DNA
tggcaccatacgaaatattc

SEQ ID NO: 416 - DNA, 18 bp, synthetic construct
  misc_feature 1..18: note = Description of Artificial Sequence: Synthetic primer
  source 1..18: mol_type = other DNA
ccggatcagtgcataaca

SEQ ID NO: 417 - DNA, 22 bp, synthetic construct
  misc_feature 1..22: note = Description of Artificial Sequence: Synthetic primer
  source 1..22: mol_type = other DNA
atcatgactgatatggtagaca

SEQ ID NO: 418 - DNA, 23 bp, synthetic construct
  misc_feature 1..23: note = Description of Artificial Sequence: Synthetic primer
  source 1..23: mol_type = other DNA
tctggagagagaacaaataaatg

SEQ ID NO: 419 - DNA, 17 bp, synthetic construct
  misc_feature 1..17: note = Description of Artificial Sequence: Synthetic primer
  source 1..17: mol_type = other DNA
actcagcctgtttctgg

SEQ ID NO: 420 - DNA, 20 bp, synthetic construct
  misc_feature 1..20: note = Description of Artificial Sequence: Synthetic primer
  source 1..20: mol_type = other DNA
cctgacagacaataaaaggc

SEQ ID NO: 421 - DNA, 20 bp, synthetic construct
  misc_feature 1..20: note = Description of Artificial Sequence: Synthetic primer
  source 1..20: mol_type = other DNA
gcttgataggtaggtactca

SEQ ID NO: 422 - DNA, 20 bp, synthetic construct
  misc_feature 1..20: note = Description of Artificial Sequence: Synthetic primer
  source 1..20: mol_type = other DNA
catgcaaattttgctgaagt

SEQ ID NO: 423 - DNA, 22 bp, synthetic construct
  misc_feature 1..22: note = Description of Artificial Sequence: Synthetic primer
  source 1..22: mol_type = other DNA
ccttccttgatcatcttgtaga

SEQ ID NO: 424 - DNA, 21 bp, synthetic construct
  misc_feature 1..21: note = Description of Artificial Sequence: Synthetic primer
  source 1..21: mol_type = other DNA
agttaaggactctgaagatgt

SEQ ID NO: 425 - DNA, 24 bp, synthetic construct
  misc_feature 1..24: note = Description of Artificial Sequence: Synthetic primer
  source 1..24: mol_type = other DNA
gtgtgacatgttctaatatagtca

SEQ ID NO: 426 - DNA, 18 bp, synthetic construct
  misc_feature 1..18: note = Description of Artificial Sequence: Synthetic primer
  source 1..18: mol_type = other DNA
gctccatgcagatactga

SEQ ID NO: 427 - DNA, 16 bp, synthetic construct
  misc_feature 1..16: note = Description of Artificial Sequence: Synthetic primer
  source 1..16: mol_type = other DNA
cctggcacccaaacat

SEQ ID NO: 428 - DNA, 19 bp, synthetic construct
  misc_feature 1..19: note = Description of Artificial Sequence: Synthetic primer
  source 1..19: mol_type = other DNA
gcttcccaaacacttagac

SEQ ID NO: 429 - DNA, 18 bp, synthetic construct
  misc_feature 1..18: note = Description of Artificial Sequence: Synthetic primer
  source 1..18: mol_type = other DNA
aagcagtgctcatgattg

SEQ ID NO: 430 - DNA, 17 bp, synthetic construct
  misc_feature 1..17: note = Description of Artificial Sequence: Synthetic primer
  source 1..17: mol_type = other DNA
ttgggcttacacttcgg

SEQ ID NO: 431 - DNA, 22 bp, synthetic construct
  misc_feature 1..22: note = Description of Artificial Sequence: Synthetic primer
  source 1..22: mol_type = other DNA
aaccacaaaagtatactccatg

SEQ ID NO: 432 - DNA, 16 bp, synthetic construct
  misc_feature 1..16: note = Description of Artificial Sequence: Synthetic primer
  source 1..16: mol_type = other DNA
ggatggctggcttaca

SEQ ID NO: 433 - DNA, 20 bp, synthetic construct
  misc_feature 1..20: note = Description of Artificial Sequence: Synthetic primer
  source 1..20: mol_type = other DNA
catctgacttggtggtaaac

SEQ ID NO: 434 - DNA, 16 bp, synthetic construct
  misc_feature 1..16: note = Description of Artificial Sequence: Synthetic primer
  source 1..16: mol_type = other DNA
cggagcttcctgagtg

SEQ ID NO: 435 - DNA, 17 bp, synthetic construct
  misc_feature 1..17: note = Description of Artificial Sequence: Synthetic primer
  source 1..17: mol_type = other DNA
gcccctctctgattgtc

SEQ ID NO: 436 - DNA, 16 bp, synthetic construct
  misc_feature 1..16: note = Description of Artificial Sequence: Synthetic primer
  source 1..16: mol_type = other DNA
ggtggtggtgctgatg

SEQ ID NO: 437 - DNA, 19 bp, synthetic construct
  misc_feature 1..19: note = Description of Artificial Sequence: Synthetic primer
  source 1..19: mol_type = other DNA
cgccaattaaccctgatta

SEQ ID NO: 438 - DNA, 21 bp, synthetic construct
  misc_feature 1..21: note = Description of Artificial Sequence: Synthetic primer
  source 1..21: mol_type = other DNA
ggatttaagcctgattgaaca

SEQ ID NO: 439 - DNA, 17 bp, synthetic construct
  misc_feature 1..17: note = Description of Artificial Sequence: Synthetic primer
  source 1..17: mol_type = other DNA
accagtgagggaagtga

SEQ ID NO: 440 - DNA, 20 bp, synthetic construct
  misc_feature 1..20: note = Description of Artificial Sequence: Synthetic primer
  source 1..20: mol_type = other DNA
ggtaaatggacaagaacact

SEQ ID NO: 441 - DNA, 18 bp, synthetic construct
  misc_feature 1..18: note = Description of Artificial Sequence: Synthetic primer
  source 1..18: mol_type = other DNA
gcccagttccctttctac

SEQ ID NO: 442 - DNA, 19 bp, synthetic construct
  misc_feature 1..19: note = Description of Artificial Sequence: Synthetic primer
  source 1..19: mol_type = other DNA
tctggctgcgagttataat

SEQ ID NO: 443 - DNA, 18 bp, synthetic construct
  misc_feature 1..18: note = Description of Artificial Sequence: Synthetic primer
  source 1..18: mol_type = other DNA
cagctttgcccatgaaac

SEQ ID NO: 444 - DNA, 16 bp, synthetic construct
  misc_feature 1..16: note = Description of Artificial Sequence: Synthetic primer
  source 1..16: mol_type = other DNA
ccaggcagcggtagta

SEQ ID NO: 445 - DNA, 16 bp, synthetic construct
  misc_feature 1..16: note = Description of Artificial Sequence: Synthetic primer
  source 1..16: mol_type = other DNA
gctactggccggaaag

SEQ ID NO: 446 - DNA, 19 bp, synthetic construct
  misc_feature 1..19: note = Description of Artificial Sequence: Synthetic primer
  source 1..19: mol_type = other DNA
tcagatgtgctgttgagac

SEQ ID NO: 447 - DNA, 16 bp, synthetic construct
  misc_feature 1..16: note = Description of Artificial Sequence: Synthetic primer
  source 1..16: mol_type = other DNA
aggatggcctctgtct

SEQ ID NO: 448 - DNA, 18 bp, synthetic construct
  misc_feature 1..18: note = Description of Artificial Sequence: Synthetic primer
  source 1..18: mol_type = other DNA
gagcaacacccacactta

SEQ ID NO: 449 - DNA, 16 bp, synthetic construct
  misc_feature 1..16: note = Description of Artificial Sequence: Synthetic primer
  source 1..16: mol_type = other DNA
cagctggccttaccat

SEQ ID NO: 450 - DNA, 17 bp, synthetic construct
  misc_feature 1..17: note = Description of Artificial Sequence: Synthetic primer
  source 1..17: mol_type = other DNA
gtagctgtgcatgtcct

SEQ ID NO: 451 - DNA, 18 bp, synthetic construct
  misc_feature 1..18: note = Description of Artificial Sequence: Synthetic primer
  source 1..18: mol_type = other DNA
ggaggtgggtgtctttat

SEQ ID NO: 452 - DNA, 16 bp, synthetic construct
  misc_feature 1..16: note = Description of Artificial Sequence: Synthetic primer
  source 1..16: mol_type = other DNA
gtcgtgggacacagtg

SEQ ID NO: 453 - DNA, 17 bp, synthetic construct
  misc_feature 1..17: note = Description of Artificial Sequence: Synthetic primer
  source 1..17: mol_type = other DNA
ggtgcgggagtgaatag

SEQ ID NO: 454 - DNA, 16 bp, synthetic construct
  misc_feature 1..16: note = Description of Artificial Sequence: Synthetic primer
  source 1..16: mol_type = other DNA
ggagggtgcagtgttg

SEQ ID NO: 455 - DNA, 19 bp, synthetic construct
  misc_feature 1..19: note = Description of Artificial Sequence: Synthetic primer
  source 1..19: mol_type = other DNA
ctccagaagcttgaactct

SEQ ID NO: 456 - DNA, 16 bp, synthetic construct
  misc_feature 1..16: note = Description of Artificial Sequence: Synthetic primer
  source 1..16: mol_type = other DNA
ctagcacgtgcctacc

SEQ ID NO: 457 - DNA, 20 bp, synthetic construct
  misc_feature 1..20: note = Description of Artificial Sequence: Synthetic primer
  source 1..20: mol_type = other DNA
cctgagtgtagatgatgtca

SEQ ID NO: 458 - DNA, 23 bp, synthetic construct
  misc_feature 1..23: note = Description of Artificial Sequence: Synthetic primer
  source 1..23: mol_type = other DNA
actcaggtactgtgtatatactt

SEQ ID NO: 459 - DNA, 18 bp, synthetic construct
  misc_feature 1..18: note = Description of Artificial Sequence: Synthetic primer
  source 1..18: mol_type = other DNA
gaagagaatctccgcaag

SEQ ID NO: 460 - DNA, 17 bp, synthetic construct
  misc_feature 1..17: note = Description of Artificial Sequence: Synthetic primer
  source 1..17: mol_type = other DNA
gcactggcctcatcttg

SEQ ID NO: 461 - DNA, 18 bp, synthetic construct
  misc_feature 1..18: note = Description of Artificial Sequence: Synthetic primer
  source 1..18: mol_type = other DNA
gccctgactttcaactct

SEQ ID NO: 462 - DNA, 16 bp, synthetic construct
  misc_feature 1..16: note = Description of Artificial Sequence: Synthetic primer
  source 1..16: mol_type = other DNA
agcgctgctcagatag

SEQ ID NO: 463 - DNA, 17 bp, synthetic construct
  misc_feature 1..17: note = Description of Artificial Sequence: Synthetic primer
  source 1..17: mol_type = other DNA
acccaggtccagatgaa

SEQ ID NO: 464 - DNA, 19 bp, synthetic construct
  misc_feature 1..19: note = Description of Artificial Sequence: Synthetic primer
  source 1..19: mol_type = other DNA
actgactttctgctcttgt